European Patent Specification EP 3 630 980 B1, published November 1, 2023. Title: Chimeric Antigen Receptor Cell Preparation and Uses thereof. Applicant: Innovative Cellular Therapeutics CO., LTD. Xiao, Lei Pu, Chengfei Cao, Zhiyuan Wu, Zhao. The sequence listing filed with the application follows.

SEQUENCE LISTING (96 sequences)

SEQ ID NO: 1 - DNA, 231 bp, Artificial Sequence
  synthesis
cggctccggtgcccgtcagtgggcagagcgcacatcgcccacagtccccgagaagttggggggaggggtcggcaattgaaccggtgcctagagaaggtggcgcggggtaaactgggaaagtgatgtcgtgtactggctccgcctttttcccgagggtgggggagaaccgtatataagtgcagtagtcgccgtgaacgttctttttcgcaacgggtttgccgccagaacaca

SEQ ID NO: 2 - DNA, 1131 bp, Artificial Sequence
  synthesis
atggcttcgtacccctgccatcaacacgcgtctgcgttcgaccaggctgcgcgttctcgcggccatagcaaccgacgtacggcgttgcgccctcgccggcagcaagaagccacggaagtccgcccggagcagaaaatgcccacgctactgcgggtttatatagacggtccccacgggatggggaaaaccaccaccacgcaactgctggtggccctgggttcgcgcgacgatatcgtctacgtacccgagccgatgacttactggcgggtgctgggggcttccgagacaatcgcgaacatctacaccacacaacaccgcctcgaccagggtgagatatcggccggggacgcggcggtggtaatgacaagcgcccagataacaatgggcatgccttatgccgtgaccgacgccgttctggctcctcatatcgggggggaggctgggagctcacatgccccgcccccggccctcaccctcatcttcgaccgccatcccatcgccgccctcctgtgctacccggccgcgcgataccttatgggcagcatgaccccccaggccgtgctggcgttcgtggccctcatcccgccgaccttgcccggcacaaacatcgtgttgggggcccttccggaggacagacacatcgaccgcctggccaaacgccagcgccccggcgagcggcttgacctggctatgctggccgcgattcgccgcgtttacgggctgcttgccaatacggtgcggtatctgcagggcggcgggtcgtggcgggaggattggggacagctttcggggacggccgtgccgccccagggtgccgagccccagagcaacgcgggcccacgaccccatatcggggacacgttatttaccctgtttcgggcccccgagttgctggcccccaacggcgacctgtataacgtgtttgcctgggccttggacgtcttggccaaacgcctccgtcccatgcacgtctttatcctggattacgaccaatcgcccgccggctgccgggacgccctgctgcaacttacctccgggatggtccagacccacgtcaccaccccaggctccataccgacgatctgcgacctggcgcgcacgtttgcccgggagatgggggaggctaactga

SEQ ID NO: 3 - DNA, 585 bp, Artificial Sequence
  synthesis
cctctccctcccccccccctaacgttactggccgaagccgcttggaataaggccggtgtgcgtttgtctatatgttattttccaccatattgccgtcttttggcaatgtgagggcccggaaacctggccctgtcttcttgacgagcattcctaggggtctttcccctctcgccaaaggaatgcaaggtctgttgaatgtcgtgaaggaagcagttcctctggaagcttcttgaagacaaacaacgtctgtagcgaccctttgcaggcagcggaaccccccacctggcgacaggtgcctctgcggccaaaagccacgtgtataagatacacctgcaaaggcggcacaaccccagtgccacgttgtgagttggatagttgtggaaagagtcaaatggctctcctcaagcgtattcaacaaggggctgaaggatgcccagaaggtaccccattgtatgggatctgatctggggcctcggtacacatgctttacatgtgtttagtcgaggttaaaaaaacgtctaggccccccgaaccacggggacgtggttttcctttgaaaaacacgatgataatatggccacaacc

SEQ ID NO: 4 - DNA, 1008 bp, Artificial Sequence
  synthesis
atgtctagattagataaaagtaaagtgattaacagcgcattagagctgcttaatgaggtcggaatcgaaggtttaacaacccgtaaactcgcccagaagcttggtgtagagcagcctacactgtattggcatgtaaaaaataagcgggctttgctcgacgccttagccattgagatgttagataggcaccatactcacttttgccctttaaaaggggaaagctggcaagattttttacgcaataacgctaaaagttttagatgtgctttactaagtcatcgcaatggagcaaaagtacattcagatacacggcctacagaaaaacagtatgaaactctcgaaaatcaattagcctttttatgccaacaaggtttttcactagagaacgcgttatatgcactcagcgctgtggggcattttactttaggttgcgtattggaagatcaagagcatcaagtcgctaaagaagaaagggaaacacctactactgatagtatgccgccattattacgacaagctatcgaattatttgatcaccaaggtgcagagccagccttcttattcggccttgaattgatcatatgcggattagaaaaacaacttaaatgtgaaagtgggtccgcgtacagccgcgcgcgtacgaaaaacaattacgggtctaccatcgagggcctgctcgatctcccggacgacgacgcccccgaagaggcggggctggcggctccgcgcctgtcctttctccccgcgggacacacgcgcagactgtcgacggcccccccgaccgatgtcagcctgggggacgagctccacttagacggcgaggacgtggcgatggcgcatgccgacgcgctagacgatttcgatctggacatgttgggggacggggattccccgggtccgggatttaccccccacgactccgccccctacggcgctctggatatggccgacttcgagtttgagcagatgtttaccgatgcccttggaattgacgagtacggtgggtag

SEQ ID NO: 5 - DNA, 438 bp, Artificial Sequence
  synthesis
ctcgagtttaccactccctatcagtgatagagaaaagtgaaagtcgagtttaccactccctatcagtgatagagaaaagtgaaagtcgagtttaccactccctatcagtgatagagaaaagtgaaagtcgagtttaccactccctatcagtgatagagaaaagtgaaagtcgagtttaccactccctatcagtgatagagaaaagtgaaagtcgagtttaccactccctatcagtgatagagaaaagtgaaagtcgagtttaccactccctatcagtgatagagaaaagtgaaagtcgagctcggtacccgggtcgagtaggcgtgtacggtgggaggcctatataagcagagctcgtttagtgaaccgtcagatcgcctggagacgccatccacgctgttttgacctccatagaagacaccgggaccgatccagcct

SEQ ID NO: 6 - DNA, 3399 bp, Artificial Sequence
  synthesis
atgccgcgcgctccccgctgccgagccgtgcgctccctgctgcgcagccactaccgcgaggtgctgccgctggccacgttcgtgcggcgcctggggccccagggctggcggctggtgcagcgcggggacccggcggctttccgcgcgctggtggcccagtgcctggtgtgcgtgccctgggacgcacggccgccccccgccgccccctccttccgccaggtgtcctgcctgaaggagctggtggcccgagtgctgcagaggctgtgcgagcgcggcgcgaagaacgtgctggccttcggcttcgcgctgctggacggggcccgcgggggcccccccgaggccttcaccaccagcgtgcgcagctacctgcccaacacggtgaccgacgcactgcgggggagcggggcgtgggggctgctgctgcgccgcgtgggcgacgacgtgctggttcacctgctggcacgctgcgcgctctttgtgctggtggctcccagctgcgcctaccaggtgtgcgggccgccgctgtaccagctcggcgctgccactcaggcccggcccccgccacacgctagtggaccccgaaggcgtctgggatgcgaacgggcctggaaccatagcgtcagggaggccggggtccccctgggcctgccagccccgggtgcgaggaggcgcgggggcagtgccagccgaagtctgccgttgcccaagaggcccaggcgtggcgctgcccctgagccggagcggacgcccgttgggcaggggtcctgggcccacccgggcaggacgcgtggaccgagtgaccgtggtttctgtgtggtgtcacctgccagacccgccgaagaagccacctctttggagggtgcgctctctggcacgcgccactcccacccatccgtgggccgccagcaccacgcgggccccccatccacatcgcggccaccacgtccctgggacacgccttgtcccccggtgtacgccgagaccaagcacttcctctactcctcaggcgacaaggagcagctgcggccctccttcctactcagctctctgaggcccagcctgactggcgctcggaggctcgtggagaccatctttctgggttccaggccctggatgccagggactccccgcaggttgccccgcctgccccagcgctactggcaaatgcggcccctgtttctggagctgcttgggaaccacgcgcagtgcccctacggggtgctcctcaagacgcactgcccgctgcgagctgcggtcaccccagcagccggtgtctgtgcccgggagaagccccagggctctgtggcggcccccgaggaggaggacacagacccccgtcgcctggtgcagctgctccgccagcacagcagcccctggcaggtgtacggcttcgtgcgggcctgcctgcgccggctggtgcccccaggcctctggggctccaggcacaacgaacgccgcttcctcaggaacaccaagaagttcatctccctggggaagcatgccaagctctcgctgcaggagctgacgtggaagatgagcgtgcgggactgcgcttggctgcgcaggagcccaggggttggctgtgttccggccgcagagcaccgtctgcgtgaggagatcctggccaagttcctgcactggctgatgagtgtgtacgtcgtcgagctgctcaggtctttcttttatgtcacggagaccacgtttcaaaagaacaggctctttttctaccggaagagtgtctggagcaagttgcaaagcattggaatcagacagcacttgaagagggtgcagctgcgggagctgtcggaagcagaggtcaggcagcatcgggaagccaggcccgccctgctgacgtccagactccgcttcatccccaagcctgacgggctgcggccgattgtgaacatggactacgtcgtgggagccagaacgttccgcagagaaaagagggccgagcgtctcacctcgagggtgaaggcactgttcagcgtgctcaactacgagcgggcgcggcgccccggcctcctgggcgcctctgtgctgggcctggacgatatccacagggcctggcgcaccttcgtgctgcgtgtgcgggcccaggacccgccgcctgagctgtactttgtcaaggtggatgtgacgggcgcgtacgacaccatcccccaggacaggctcacggaggtcatcgccagcatcatcaaaccccagaacacgtactgcgtgcgtcggtatgccgtggtccagaaggccgcccatgggcacgtccgcaaggccttcaagagccacgtctctaccttgacagacctccagccgtacatgcgacagttcgtggctcacctgcaggagaccagcccgctgagggatgccgtcgtcatcgagcagagctcctccctgaatgaggccagcagtggcctcttcgacgtcttcctacgcttcatgtgccaccacgccgtgcgcatcaggggcaagtcctacgtccagtgccaggggatcccgcagggctccatcctctccacgctgctctgcagcctgtgctacggcgacatggagaacaagctgtttgcggggattcggcgggacgggctgctcctgcgtttggtggatgatttcttgttggtgacacctcacctcacccacgcgaaaaccttcctcaggaccctggtccgaggtgtccctgagtatggctgcgtggtgaacttgcggaagacagtggtgaacttccctgtagaagacgaggccctgggtggcacggcttttgttcagatgccggcccacggcctattcccctggtgcggcctgctgctggatacccggaccctggaggtgcagagcgactactccagctatgcccggacctccatcagagccagtctcaccttcaaccgcggcttcaaggctgggaggaacatgcgtcgcaaactctttggggtcttgcggctgaagtgtcacagcctgtttctggatttgcaggtgaacagcctccagacggtgtgcaccaacatctacaagatcctcctgctgcaggcgtacaggtttcacgcatgtgtgctgcagctcccatttcatcagcaagtttggaagaaccccacatttttcctgcgcgtcatctctgacacggcctccctctgctactccatcctgaaagccaagaacgcagggatgtcgctgggggccaagggcgccgccggccctctgccctccgaggccgtgcagtggctgtgccaccaagcattcctgctcaagctgactcgacaccgtgtcacctacgtgccactcctggggtcactcaggacagcccagacgcagctgagtcggaagctcccggggacgacgctgactgccctggaggccgcagccaacccggcactgccctcagacttcaagaccatcctggactga

SEQ ID NO: 7 - DNA, 2127 bp, Artificial Sequence
  synthesis
atggataaagttttaaacagagaggaatctttgcagctaatggaccttctaggtcttgaaaggagtgcctgggggaatattcctctgatgagaaaggcatatttaaaaaaatgcaaggagtttcatcctgataaaggaggagatgaagaaaaaatgaagaaaatgaatactctgtacaagaaaatggaagatggagtaaaatatgctcatcaacctgactttggaggcttctgggatgcaactgagattccaacctatggaactgatgaatgggagcagtggtggaatgcctttaatgaggaaaacctgttttgctcagaagaaatgccatctagtgatgatgaggctactgctgactctcaacattctactcctccaaaaaagaagagaaaggtagaagaccccaaggactttccttcagaattgctaagttttttgagtcatgctgtgtttagtaatagaactcttgcttgctttgctatttacaccacaaaggaaaaagctgcactgctatacaagaaaattatggaaaaatattctgtaacctttataagtaggcataacagttataatcataacatactgttttttcttactccacacaggcatagagtgtctgctattaataactatgctcaaaaattgtgtacctttagctttttaatttgtaaaggggttaataaggaatatttgatgtatagtgccttgactagagatccattttctgttattgaggaaagtttgccaggtgggttaaaggagcatgattttaatccagaagaagcagaggaaactaaacaagtgtcctggaagcttgtaacagagtatgcaatggaaacaaaatgtgatgatgtgttgttattgcttgggatgtacttggaatttcagtacagttttgaaatgtgtttaaaatgtattaaaaaagaacagcccagccactataagtaccatgaaaagcattatgcaaatgctgctatatttgctgacagcaaaaaccaaaaaaccatatgccaacaggctgttgatactgttttagctaaaaagcgggttgatagcctacaattaactagagaacaaatgttaacaaacagatttaatgatcttttggataggatggatataatgtttggttctacaggctctgctgacatagaagaatggatggctggagttgcttggctacactgtttgttgcccaaaatggattcagtggtgtatgactttttaaaatgcatggtgtacaacattcctaaaaaaagatactggctgtttaaaggaccaattgatagtggtaaaactacattagcagctgctttgcttgaattatgtggggggaaagctttaaatgttaatttgcccttggacaggctgaactttgagctaggagtagctattgaccagtttttagtagtttttgaggatgtaaagggcactggaggggagtccagagatttgccttcaggtcagggaattaataacctggacaatttaagggattatttggatggcagtgttaaggtaaacttagaaaagaaacacctaaataaaagaactcaaatatttccccctggaatagtcaccatgaatgagtacagtgtgcctaaaacactgcaggccagatttgtaaaacaaatagattttaggcccaaagattatttaaagcattgcctggaacgcagtgagtttttgttagaaaagagaataattcaaagtggcattgctttgcttcttatgttaatttggtacagacctgtggctgagtttgctcaaagtattcagagcagaattgtggagtggaaagagagattggacaaagagtttagtttgtcagtgtatcaaaaaatgaagtttaatgtggctatgggaattggagttttagattggctaagaaacagtgatgatgatgatgaagacagccaggaaaatgctgataaaaatgaagatggtggggagaagaacatggaagactcagggcatgaaacaggcattgattcacagtcccaaggctcatttcaggcccctcagtcctcacagtctgttcatgatcataatcagccataccacatttgtagaggttttacttgctttaaaaaacctcccacacctccccctgaacctgaaacataa

SEQ ID NO: 8 - DNA, 7902 bp, Artificial Sequence
  synthesis
gtcgacactagtaatcaacctctggattacaaaatttgtgaaagattgactggtattcttaactatgttgctccttttacgctatgtggatacgctgctttaatgcctttgtatcatgctattgcttcccgtatggctttcattttctcctccttgtataaatcctggttgctgtctctttatgaggagttgtggcccgttgtcaggcaacgtggcgtggtgtgcactgtgtttgctgacgcaacccccactggttggggcattgccaccacctgtcagctcctttccgggactttcgctttccccctccctattgccacggcggaactcatcgccgcctgccttgcccgctgctggacaggggctcggctgttgggcactgacaattccgtggtgttgtcggggaagctgacgtcctttccatggctgctcgcctgtgttgccacctggattctgcgcgggacgtccttctgctacgtcccttcggccctcaatccagcggaccttccttcccgcggcctgctgccggctctgcggcctcttccgcgtcttcgccttcgccctcagacgagtcggatctccctttgggccgcctccccgcctgccgcggaattcgagctcggtacctttaagaccaatgacttacaaggcagctgtagatcttagccactttttaaaagaaaaggggggactggaagggctaattcactcccaacgaagacaagatctgctttttgcttgtactgagtctctctggttagaccagatctgagcctgggagctctctggctaactagggaacccactgcttaagcctcaataaagcttgccttgagtgcttcaagtagtgtgtgcccgtctgttgtgtgactctggtaactagagatccctcagacccttttagtcagtgtggaaaatctctagcagtagtagttcatgtcatcttattattcagtatttataacttgcaaagaaatgaatatcagagagtgagaggaacttgtttattgcagcttataatggttacaaataaagcaatagcatcacaaatttcacaaataaagcatttttttcactgcattctagttgtggtttgtccaaactcatcaatgtatcttatcatgtctggctctagctatcccgcccctaactccgcccatcccgcccctaactccgcccagttccgcccattctccgccccatggctgactaattttttttatttatgcagaggccgaggccgcctcggcctctgagctattccagaagtagtgaggaggcttttttggaggcctagggacgtacccaattcgccctatagtgagtcgtattacgcgcgctcactggccgtcgttttacaacgtcgtgactgggaaaaccctggcgttacccaacttaatcgccttgcagcacatccccctttcgccagctggcgtaatagcgaagaggcccgcaccgatcgcccttcccaacagttgcgcagcctgaatggcgaatgggacgcgccctgtagcggcgcattaagcgcggcgggtgtggtggttacgcgcagcgtgaccgctacacttgccagcgccctagcgcccgctcctttcgctttcttcccttcctttctcgccacgttcgccggctttccccgtcaagctctaaatcgggggctccctttagggttccgatttagtgctttacggcacctcgaccccaaaaaacttgattagggtgatggttcacgtagtgggccatcgccctgatagacggtttttcgccctttgacgttggagtccacgttctttaatagtggactcttgttccaaactggaacaacactcaaccctatctcggtctattcttttgatttataagggattttgccgatttcggcctattggttaaaaaatgagctgatttaacaaaaatttaacgcgaattttaacaaaatattaacgcttacaatttaggtggcacttttcggggaaatgtgcgcggaacccctatttgtttatttttctaaatacattcaaatatgtatccgctcatgagacaataaccctgataaatgcttcaataatattgaaaaaggaagagtatgagtattcaacatttccgtgtcgcccttattcccttttttgcggcattttgccttcctgtttttgctcacccagaaacgctggtgaaagtaaaagatgctgaagatcagttgggtgcacgagtgggttacatcgaactggatctcaacagcggtaagatccttgagagttttcgccccgaagaacgttttccaatgatgagcacttttaaagttctgctatgtggcgcggtattatcccgtattgacgccgggcaagagcaactcggtcgccgcatacactattctcagaatgacttggttgagtactcaccagtcacagaaaagcatcttacggatggcatgacagtaagagaattatgcagtgctgccataaccatgagtgataacactgcggccaacttacttctgacaacgatcggaggaccgaaggagctaaccgcttttttgcacaacatgggggatcatgtaactcgccttgatcgttgggaaccggagctgaatgaagccataccaaacgacgagcgtgacaccacgatgcctgtagcaatggcaacaacgttgcgcaaactattaactggcgaactacttactctagcttcccggcaacaattaatagactggatggaggcggataaagttgcaggaccacttctgcgctcggcccttccggctggctggtttattgctgataaatctggagccggtgagcgtggctctcgcggtatcattgcagcactggggccagatggtaagccctcccgtatcgtagttatctacacgacggggagtcaggcaactatggatgaacgaaatagacagatcgctgagataggtgcctcactgattaagcattggtaactgtcagaccaagtttactcatatatactttagattgatttaaaacttcatttttaatttaaaaggatctaggtgaagatcctttttgataatctcatgaccaaaatcccttaacgtgagttttcgttccactgagcgtcagaccccgtagaaaagatcaaaggatcttcttgagatcctttttttctgcgcgtaatctgctgcttgcaaacaaaaaaaccaccgctaccagcggtggtttgtttgccggatcaagagctaccaactctttttccgaaggtaactggcttcagcagagcgcagataccaaatactgttcttctagtgtagccgtagttaggccaccacttcaagaactctgtagcaccgcctacatacctcgctctgctaatcctgttaccagtggctgctgccagtggcgataagtcgtgtcttaccgggttggactcaagacgatagttaccggataaggcgcagcggtcgggctgaacggggggttcgtgcacacagcccagcttggagcgaacgacctacaccgaactgagatacctacagcgtgagctatgagaaagcgccacgcttcccgaagggagaaaggcggacaggtatccggtaagcggcagggtcggaacaggagagcgcacgagggagcttccagggggaaacgcctggtatctttatagtcctgtcgggtttcgccacctctgacttgagcgtcgatttttgtgatgctcgtcaggggggcggagcctatggaaaaacgccagcaacgcggcctttttacggttcctggccttttgctggccttttgctcacatgttctttcctgcgttatcccctgattctgtggataaccgtattaccgcctttgagtgagctgataccgctcgccgcagccgaacgaccgagcgcagcgagtcagtgagcgaggaagcggaagagcgcccaatacgcaaaccgcctctccccgcgcgttggccgattcattaatgcagctggcacgacaggtttcccgactggaaagcgggcagtgagcgcaacgcaattaatgtgagttagctcactcattaggcaccccaggctttacactttatgcttccggctcgtatgttgtgtggaattgtgagcggataacaatttcacacaggaaacagctatgaccatgattacgccaagcgcgcaattaaccctcactaaagggaacaaaagctggagctgcaagcttaatgtagtcttatgcaatactcttgtagtcttgcaacatggtaacgatgagttagcaacatgccttacaaggagagaaaaagcaccgtgcatgccgattggtggaagtaaggtggtacgatcgtgccttattaggaaggcaacagacgggtctgacatggattggacgaaccactgaattgccgcattgcagagatattgtatttaagtgcctagctcgatacataaacggctctctctggttagaccagatctgagcctgggagctctctggctaactagggaacccactgcttaagcctcaataaagcttgccttgagtgcttcaagtagtgtgtgcccgtctgttgtgtgactctggtaactagagatccctcagacccttttagtcagtgtggaaaatctctagcagtggcgcccgaacagggacttgaaagcgaaagggaaaccagaggagctctctcgacgcaggactcggcttgctgaagcgcgcacggcaagaggcgaggggcggcgactggtgagtacgccaaaaattttgactagcggaggctagaaggagagagatgggtgcgagagcgtcagtattaagcgggggagaattagatcgcgatgggaaaaaattcggttaaggccagggggaaagaaaaaatataaattaaaacatatagtatgggcaagcagggagctagaacgattcgcagttaatcctggcctgttagaaacatcagaaggctgtagacaaatactgggacagctacaaccatcccttcagacaggatcagaagaacttagatcattatataatacagtagcaaccctctattgtgtgcatcaaaggatagagataaaagacaccaaggaagctttagacaagatagaggaagagcaaaacaaaagtaagaccaccgcacagcaagcggccgctgatcttcagacctggaggaggagatatgagggacaattggagaagtgaattatataaatataaagtagtaaaaattgaaccattaggagtagcacccaccaaggcaaagagaagagtggtgcagagagaaaaaagagcagtgggaataggagctttgttccttgggttcttgggagcagcaggaagcactatgggcgcagcgtcaatgacgctgacggtacaggccagacaattattgtctggtatagtgcagcagcagaacaatttgctgagggctattgaggcgcaacagcatctgttgcaactcacagtctggggcatcaagcagctccaggcaagaatcctggctgtggaaagatacctaaaggatcaacagctcctggggatttggggttgctctggaaaactcatttgcaccactgctgtgccttggaatgctagttggagtaataaatctctggaacagatttggaatcacacgacctggatggagtgggacagagaaattaacaattacacaagcttaatacactccttaattgaagaatcgcaaaaccagcaagaaaagaatgaacaagaattattggaattagataaatgggcaagtttgtggaattggtttaacataacaaattggctgtggtatataaaattattcataatgatagtaggaggcttggtaggtttaagaatagtttttgctgtactttctatagtgaatagagttaggcagggatattcaccattatcgtttcagacccacctcccaaccccgaggggacccgacaggcccgaaggaatagaagaagaaggtggagagagagacagagacagatccattcgattagtgaacggatctcgacggtatcgatcacgagactagcctcgacacaaatggcagtattcatccacaattttaaaagaaaaggggggattggggggtacagtgcaggggaaagaatagtagacataatagcaacagacatacaaactaaagaattacaaaaacaaattacaaaaattcaaaattttcgggtttattacagggacagcagaaatccactttggctcgagaagcttgatatcggctccggtgcccgtcagtgggcagagcgcacatcgcccacagtccccgagaagttggggggaggggtcggcaattgaaccggtgcctagagaaggtggcgcggggtaaactgggaaagtgatgtcgtgtactggctccgcctttttcccgagggtgggggagaaccgtatataagtgcagtagtcgccgtgaacgttctttttcgcaacgggtttgccgccagaacacaggatccgccaccatggccttaccagtgaccgccttgctcctgccgctggccttgctgctccacgccgccaggccggatatccagatgacccagagcccgagcagcctgagcgcgagcgtgggtgatcgcgtgaccattacctgcagggcaagtcaggacattagtaaatatttaaattggtatcagcagaaaccgggtaaagcgccgaaactgttaatttatcatacatcaagattacactcaggcgtgccgtcgcgttttagcggctcgggttcgggcaccgattttaccctgaccatctcgagcttgcagccggaggacttcgccacctactattgccaacagggtaatacgcttccgtacacgttcggtcagggcaccaaagtggagatcaaaggtggcggtggctcgggcggtggtgggtcgggtggcggcggatctgaggtgcagctggtggagtctgggggaggcttggtacagcctggggggtccctgagactctcctgtgcagcctctggagtgtccctgcctgattatggcgtgtcctgggtccgccaggctccagggaaggggctggagtgggtttcagtgatctggggcagcgagacaacctactacaacagcgccctgaagtcccgattcaccatctccagagacaatgccaagaactcactgtatctgcaaatgaacagcctgagagccgaggacacggctgtgtattactgtgcgaagcactactactacggcggcagctacgctatggactactggggccaaggaaccctggtcaccgtgtcctcaaccacgacgccagcgccgcgaccaccaacaccggcgcccaccatcgcgtcgcagcccctgtccctgcgcccagaggcgtgccggccagcggcggggggcgcagtgcacacgagggggctggacttcgcctgtgatatctacatctgggcgcccttggccgggacttgtggggtccttctcctgtcactggttatcaccctttactgcaaacggggcagaaagaaactcctgtatatattcaaacaaccatttatgagaccagtacaaactactcaagaggaagatggctgtagctgccgatttccagaagaagaagaaggaggatgtgaactgagagtgaagttcagcaggagcgcagacgcccccgcgtacaagcagggccagaaccagctctataacgagctcaatctaggacgaagagaggagtacgatgttttggacaagaggcgtggccgggaccctgagatggggggaaagccgagaaggaagaaccctcaggaaggcctgtacaatgaactgcagaaagataagatggcggaggcctacagtgagattgggatgaaaggcgagcgccggaggggcaaggggcacgatggcctttaccagggtctcagtacagccaccaaggacacctacgacgcccttcacatgcaggccctgccccctcgctaatctagaggcgcgcc

SEQ ID NO: 9 - DNA, 9162 bp, Artificial Sequence
  synthesis
cctctccctcccccccccctaacgttactggccgaagccgcttggaataaggccggtgtgcgtttgtctatatgttattttccaccatattgccgtcttttggcaatgtgagggcccggaaacctggccctgtcttcttgacgagcattcctaggggtctttcccctctcgccaaaggaatgcaaggtctgttgaatgtcgtgaaggaagcagttcctctggaagcttcttgaagacaaacaacgtctgtagcgaccctttgcaggcagcggaaccccccacctggcgacaggtgcctctgcggccaaaagccacgtgtataagatacacctgcaaaggcggcacaaccccagtgccacgttgtgagttggatagttgtggaaagagtcaaatggctctcctcaagcgtattcaacaaggggctgaaggatgcccagaaggtaccccattgtatgggatctgatctggggcctcggtacacatgctttacatgtgtttagtcgaggttaaaaaaacgtctaggccccccgaaccacggggacgtggttttcctttgaaaaacacgatgataatatggccacaaccatgcagatcccacaggcgccctggccagtcgtctgggcggtgctacaactgggctggcggccaggatggttcttagactccccagacaggccctggaacccccccaccttctccccagccctgctcgtggtgaccgaaggggacaacgccaccttcacctgcagcttctccaacacatcggagagcttcgtgctaaactggtaccgcatgagccccagcaaccagacggacaagctggccgccttccccgaggaccgcagccagcccggccaggactgccgcttccgtgtcacacaactgcccaacgggcgtgacttccacatgagcgtggtcagggcccggcgcaatgacagcggcacctacctctgtggggccatctccctggcccccaaggcgcagatcaaagagagcctgcgggcagagctcagggtgacagagagaagggcagaagtgcccacagcccaccccagcccctcacccaggccagccggccagttccaaaccctggtggttggtgtcgtgggcggcctgctgggcagcctggtgctgctagtctgggtcctggccgtcatctgctcccgggccgcacgagggacaatagattacaaggatgacgacgataaggattacaaggatgacgacgataaggattacaaggatgacgacgataagtaagtcgacactagtaatcaacctctggattacaaaatttgtgaaagattgactggtattcttaactatgttgctccttttacgctatgtggatacgctgctttaatgcctttgtatcatgctattgcttcccgtatggctttcattttctcctccttgtataaatcctggttgctgtctctttatgaggagttgtggcccgttgtcaggcaacgtggcgtggtgtgcactgtgtttgctgacgcaacccccactggttggggcattgccaccacctgtcagctcctttccgggactttcgctttccccctccctattgccacggcggaactcatcgccgcctgccttgcccgctgctggacaggggctcggctgttgggcactgacaattccgtggtgttgtcggggaagctgacgtcctttccatggctgctcgcctgtgttgccacctggattctgcgcgggacgtccttctgctacgtcccttcggccctcaatccagcggaccttccttcccgcggcctgctgccggctctgcggcctcttccgcgtcttcgccttcgccctcagacgagtcggatctccctttgggccgcctccccgcctgccgcggaattcgagctcggtacctttaagaccaatgacttacaaggcagctgtagatcttagccactttttaaaagaaaaggggggactggaagggctaattcactcccaacgaagacaagatctgctttttgcttgtactgagtctctctggttagaccagatctgagcctgggagctctctggctaactagggaacccactgcttaagcctcaataaagcttgccttgagtgcttcaagtagtgtgtgcccgtctgttgtgtgactctggtaactagagatccctcagacccttttagtcagtgtggaaaatctctagcagtagtagttcatgtcatcttattattcagtatttataacttgcaaagaaatgaatatcagagagtgagaggaacttgtttattgcagcttataatggttacaaataaagcaatagcatcacaaatttcacaaataaagcatttttttcactgcattctagttgtggtttgtccaaactcatcaatgtatcttatcatgtctggctctagctatcccgcccctaactccgcccatcccgcccctaactccgcccagttccgcccattctccgccccatggctgactaattttttttatttatgcagaggccgaggccgcctcggcctctgagctattccagaagtagtgaggaggcttttttggaggcctagggacgtacccaattcgccctatagtgagtcgtattacgcgcgctcactggccgtcgttttacaacgtcgtgactgggaaaaccctggcgttacccaacttaatcgccttgcagcacatccccctttcgccagctggcgtaatagcgaagaggcccgcaccgatcgcccttcccaacagttgcgcagcctgaatggcgaatgggacgcgccctgtagcggcgcattaagcgcggcgggtgtggtggttacgcgcagcgtgaccgctacacttgccagcgccctagcgcccgctcctttcgctttcttcccttcctttctcgccacgttcgccggctttccccgtcaagctctaaatcgggggctccctttagggttccgatttagtgctttacggcacctcgaccccaaaaaacttgattagggtgatggttcacgtagtgggccatcgccctgatagacggtttttcgccctttgacgttggagtccacgttctttaatagtggactcttgttccaaactggaacaacactcaaccctatctcggtctattcttttgatttataagggattttgccgatttcggcctattggttaaaaaatgagctgatttaacaaaaatttaacgcgaattttaacaaaatattaacgcttacaatttaggtggcacttttcggggaaatgtgcgcggaacccctatttgtttatttttctaaatacattcaaatatgtatccgctcatgagacaataaccctgataaatgcttcaataatattgaaaaaggaagagtatgagtattcaacatttccgtgtcgcccttattcccttttttgcggcattttgccttcctgtttttgctcacccagaaacgctggtgaaagtaaaagatgctgaagatcagttgggtgcacgagtgggttacatcgaactggatctcaacagcggtaagatccttgagagttttcgccccgaagaacgttttccaatgatgagcacttttaaagttctgctatgtggcgcggtattatcccgtattgacgccgggcaagagcaactcggtcgccgcatacactattctcagaatgacttggttgagtactcaccagtcacagaaaagcatcttacggatggcatgacagtaagagaattatgcagtgctgccataaccatgagtgataacactgcggccaacttacttctgacaacgatcggaggaccgaaggagctaaccgcttttttgcacaacatgggggatcatgtaactcgccttgatcgttgggaaccggagctgaatgaagccataccaaacgacgagcgtgacaccacgatgcctgtagcaatggcaacaacgttgcgcaaactattaactggcgaactacttactctagcttcccggcaacaattaatagactggatggaggcggataaagttgcaggaccacttctgcgctcggcccttccggctggctggtttattgctgataaatctggagccggtgagcgtggctctcgcggtatcattgcagcactggggccagatggtaagccctcccgtatcgtagttatctacacgacggggagtcaggcaactatggatgaacgaaatagacagatcgctgagataggtgcctcactgattaagcattggtaactgtcagaccaagtttactcatatatactttagattgatttaaaacttcatttttaatttaaaaggatctaggtgaagatcctttttgataatctcatgaccaaaatcccttaacgtgagttttcgttccactgagcgtcagaccccgtagaaaagatcaaaggatcttcttgagatcctttttttctgcgcgtaatctgctgcttgcaaacaaaaaaaccaccgctaccagcggtggtttgtttgccggatcaagagctaccaactctttttccgaaggtaactggcttcagcagagcgcagataccaaatactgttcttctagtgtagccgtagttaggccaccacttcaagaactctgtagcaccgcctacatacctcgctctgctaatcctgttaccagtggctgctgccagtggcgataagtcgtgtcttaccgggttggactcaagacgatagttaccggataaggcgcagcggtcgggctgaacggggggttcgtgcacacagcccagcttggagcgaacgacctacaccgaactgagatacctacagcgtgagctatgagaaagcgccacgcttcccgaagggagaaaggcggacaggtatccggtaagcggcagggtcggaacaggagagcgcacgagggagcttccagggggaaacgcctggtatctttatagtcctgtcgggtttcgccacctctgacttgagcgtcgatttttgtgatgctcgtcaggggggcggagcctatggaaaaacgccagcaacgcggcctttttacggttcctggccttttgctggccttttgctcacatgttctttcctgcgttatcccctgattctgtggataaccgtattaccgcctttgagtgagctgataccgctcgccgcagccgaacgaccgagcgcagcgagtcagtgagcgaggaagcggaagagcgcccaatacgcaaaccgcctctccccgcgcgttggccgattcattaatgcagctggcacgacaggtttcccgactggaaagcgggcagtgagcgcaacgcaattaatgtgagttagctcactcattaggcaccccaggctttacactttatgcttccggctcgtatgttgtgtggaattgtgagcggataacaatttcacacaggaaacagctatgaccatgattacgccaagcgcgcaattaaccctcactaaagggaacaaaagctggagctgcaagcttaatgtagtcttatgcaatactcttgtagtcttgcaacatggtaacgatgagttagcaacatgccttacaaggagagaaaaagcaccgtgcatgccgattggtggaagtaaggtggtacgatcgtgccttattaggaaggcaacagacgggtctgacatggattggacgaaccactgaattgccgcattgcagagatattgtatttaagtgcctagctcgatacataaacggctctctctggttagaccagatctgagcctgggagctctctggctaactagggaacccactgcttaagcctcaataaagcttgccttgagtgcttcaagtagtgtgtgcccgtctgttgtgtgactctggtaactagagatccctcagacccttttagtcagtgtggaaaatctctagcagtggcgcccgaacagggacttgaaagcgaaagggaaaccagaggagctctctcgacgcaggactcggcttgctgaagcgcgcacggcaagaggcgaggggcggcgactggtgagtacgccaaaaattttgactagcggaggctagaaggagagagatgggtgcgagagcgtcagtattaagcgggggagaattagatcgcgatgggaaaaaattcggttaaggccagggggaaagaaaaaatataaattaaaacatatagtatgggcaagcagggagctagaacgattcgcagttaatcctggcctgttagaaacatcagaaggctgtagacaaatactgggacagctacaaccatcccttcagacaggatcagaagaacttagatcattatataatacagtagcaaccctctattgtgtgcatcaaaggatagagataaaagacaccaaggaagctttagacaagatagaggaagagcaaaacaaaagtaagaccaccgcacagcaagcggccgctgatcttcagacctggaggaggagatatgagggacaattggagaagtgaattatataaatataaagtagtaaaaattgaaccattaggagtagcacccaccaaggcaaagagaagagtggtgcagagagaaaaaagagcagtgggaataggagctttgttccttgggttcttgggagcagcaggaagcactatgggcgcagcgtcaatgacgctgacggtacaggccagacaattattgtctggtatagtgcagcagcagaacaatttgctgagggctattgaggcgcaacagcatctgttgcaactcacagtctggggcatcaagcagctccaggcaagaatcctggctgtggaaagatacctaaaggatcaacagctcctggggatttggggttgctctggaaaactcatttgcaccactgctgtgccttggaatgctagttggagtaataaatctctggaacagatttggaatcacacgacctggatggagtgggacagagaaattaacaattacacaagcttaatacactccttaattgaagaatcgcaaaaccagcaagaaaagaatgaacaagaattattggaattagataaatgggcaagtttgtggaattggtttaacataacaaattggctgtggtatataaaattattcataatgatagtaggaggcttggtaggtttaagaatagtttttgctgtactttctatagtgaatagagttaggcagggatattcaccattatcgtttcagacccacctcccaaccccgaggggacccgacaggcccgaaggaatagaagaagaaggtggagagagagacagagacagatccattcgattagtgaacggatctcgacggtatcgatcacgagactagcctcgacacaaatggcagtattcatccacaattttaaaagaaaaggggggattggggggtacagtgcaggggaaagaatagtagacataatagcaacagacatacaaactaaagaattacaaaaacaaattacaaaaattcaaaattttcgggtttattacagggacagcagaaatccactttggctcgagaagcttgatatcggctccggtgcccgtcagtgggcagagcgcacatcgcccacagtccccgagaagttggggggaggggtcggcaattgaaccggtgcctagagaaggtggcgcggggtaaactgggaaagtgatgtcgtgtactggctccgcctttttcccgagggtgggggagaaccgtatataagtgcagtagtcgccgtgaacgttctttttcgcaacgggtttgccgccagaacacaggatccgccaccatggccttaccagtgaccgccttgctcctgccgctggccttgctgctccacgccgccaggccggatatccagatgacccagagcccgagcagcctgagcgcgagcgtgggtgatcgcgtgaccattacctgcagggcaagtcaggacattagtaaatatttaaattggtatcagcagaaaccgggtaaagcgccgaaactgttaatttatcatacatcaagattacactcaggcgtgccgtcgcgttttagcggctcgggttcgggcaccgattttaccctgaccatctcgagcttgcagccggaggacttcgccacctactattgccaacagggtaatacgcttccgtacacgttcggtcagggcaccaaagtggagatcaaaggtggcggtggctcgggcggtggtgggtcgggtggcggcggatctgaggtgcagctggtggagtctgggggaggcttggtacagcctggggggtccctgagactctcctgtgcagcctctggagtgtccctgcctgattatggcgtgtcctgggtccgccaggctccagggaaggggctggagtgggtttcagtgatctggggcagcgagacaacctactacaacagcgccctgaagtcccgattcaccatctccagagacaatgccaagaactcactgtatctgcaaatgaacagcctgagagccgaggacacggctgtgtattactgtgcgaagcactactactacggcggcagctacgctatggactactggggccaaggaaccctggtcaccgtgtcctcaaccacgacgccagcgccgcgaccaccaacaccggcgcccaccatcgcgtcgcagcccctgtccctgcgcccagaggcgtgccggccagcggcggggggcgcagtgcacacgagggggctggacttcgcctgtgatatctacatctgggcgcccttggccgggacttgtggggtccttctcctgtcactggttatcaccctttactgcaaacggggcagaaagaaactcctgtatatattcaaacaaccatttatgagaccagtacaaactactcaagaggaagatggctgtagctgccgatttccagaagaagaagaaggaggatgtgaactgagagtgaagttcagcaggagcgcagacgcccccgcgtacaagcagggccagaaccagctctataacgagctcaatctaggacgaagagaggagtacgatgttttggacaagaggcgtggccgggaccctgagatggggggaaagccgagaaggaagaaccctcaggaaggcctgtacaatgaactgcagaaagataagatggcggaggcctacagtgagattgggatgaaaggcgagcgccggaggggcaaggggcacgatggcctttaccagggtctcagtacagccaccaaggacacctacgacgcccttcacatgcaggccctgccccctcgctaatctagaggcgcgcc

SEQ ID NO: 10 - DNA, 9354 bp, Artificial Sequence
  synthesis
cctctccctcccccccccctaacgttactggccgaagccgcttggaataaggccggtgtgcgtttgtctatatgttattttccaccatattgccgtcttttggcaatgtgagggcccggaaacctggccctgtcttcttgacgagcattcctaggggtctttcccctctcgccaaaggaatgcaaggtctgttgaatgtcgtgaaggaagcagttcctctggaagcttcttgaagacaaacaacgtctgtagcgaccctttgcaggcagcggaaccccccacctggcgacaggtgcctctgcggccaaaagccacgtgtataagatacacctgcaaaggcggcacaaccccagtgccacgttgtgagttggatagttgtggaaagagtcaaatggctctcctcaagcgtattcaacaaggggctgaaggatgcccagaaggtaccccattgtatgggatctgatctggggcctcggtacacatgctttacatgtgtttagtcgaggttaaaaaaacgtctaggccccccgaaccacggggacgtggttttcctttgaaaaacacgatgataatatggccacaaccatgcagatcccacaggcgccctggccagtcgtctgggcggtgctacaactgggctggcggccaggatggttcttagactccccagacaggccctggaacccccccaccttctccccagccctgctcgtggtgaccgaaggggacaacgccaccttcacctgcagcttctccaacacatcggagagcttcgtgctaaactggtaccgcatgagccccagcaaccagacggacaagctggccgccttccccgaggaccgcagccagcccggccaggactgccgcttccgtgtcacacaactgcccaacgggcgtgacttccacatgagcgtggtcagggcccggcgcaatgacagcggcacctacctctgtggggccatctccctggcccccaaggcgcagatcaaagagagcctgcgggcagagctcagggtgacagagagaagggcagaagtgcccacagcccaccccagcccctcacccaggccagccggccagttccaaaccctggtggttggtgtcgtgggcggcctgctgggcagcctggtgctgctagtctgggtcctggccgtcatctgctcccgggccgcacgagggacaataggagccaggcgcaccggccagcccctgaaggaggacccctcagccgtgcctgtgttctctgtggacgccggggagctggatttccagtggcgagagaagaccccggagccccccgtgccctgtgtccctgagcagacggaggccgccaccattgtctttcctagcggaatgggcacctcatcccccgcccgcaggggctcagctgacggccctcggagtgcccagccactgaggcctgaggatggacactgctcttggcccctctgagtcgacactagtaatcaacctctggattacaaaatttgtgaaagattgactggtattcttaactatgttgctccttttacgctatgtggatacgctgctttaatgcctttgtatcatgctattgcttcccgtatggctttcattttctcctccttgtataaatcctggttgctgtctctttatgaggagttgtggcccgttgtcaggcaacgtggcgtggtgtgcactgtgtttgctgacgcaacccccactggttggggcattgccaccacctgtcagctcctttccgggactttcgctttccccctccctattgccacggcggaactcatcgccgcctgccttgcccgctgctggacaggggctcggctgttgggcactgacaattccgtggtgttgtcggggaagctgacgtcctttccatggctgctcgcctgtgttgccacctggattctgcgcgggacgtccttctgctacgtcccttcggccctcaatccagcggaccttccttcccgcggcctgctgccggctctgcggcctcttccgcgtcttcgccttcgccctcagacgagtcggatctccctttgggccgcctccccgcctgccgcggaattcgagctcggtacctttaagaccaatgacttacaaggcagctgtagatcttagccactttttaaaagaaaaggggggactggaagggctaattcactcccaacgaagacaagatctgctttttgcttgtactgagtctctctggttagaccagatctgagcctgggagctctctggctaactagggaacccactgcttaagcctcaataaagcttgccttgagtgcttcaagtagtgtgtgcccgtctgttgtgtgactctggtaactagagatccctcagacccttttagtcagtgtggaaaatctctagcagtagtagttcatgtcatcttattattcagtatttataacttgcaaagaaatgaatatcagagagtgagaggaacttgtttattgcagcttataatggttacaaataaagcaatagcatcacaaatttcacaaataaagcatttttttcactgcattctagttgtggtttgtccaaactcatcaatgtatcttatcatgtctggctctagctatcccgcccctaactccgcccatcccgcccctaactccgcccagttccgcccattctccgccccatggctgactaattttttttatttatgcagaggccgaggccgcctcggcctctgagctattccagaagtagtgaggaggcttttttggaggcctagggacgtacccaattcgccctatagtgagtcgtattacgcgcgctcactggccgtcgttttacaacgtcgtgactgggaaaaccctggcgttacccaacttaatcgccttgcagcacatccccctttcgccagctggcgtaatagcgaagaggcccgcaccgatcgcccttcccaacagttgcgcagcctgaatggcgaatgggacgcgccctgtagcggcgcattaagcgcggcgggtgtggtggttacgcgcagcgtgaccgctacacttgccagcgccctagcgcccgctcctttcgctttcttcccttcctttctcgccacgttcgccggctttccccgtcaagctctaaatcgggggctccctttagggttccgatttagtgctttacggcacctcgaccccaaaaaacttgattagggtgatggttcacgtagtgggccatcgccctgatagacggtttttcgccctttgacgttggagtccacgttctttaatagtggactcttgttccaaactggaacaacactcaaccctatctcggtctattcttttgatttataagggattttgccgatttcggcctattggttaaaaaatgagctgatttaacaaaaatttaacgcgaattttaacaaaatattaacgcttacaatttaggtggcacttttcggggaaatgtgcgcggaacccctatttgtttatttttctaaatacattcaaatatgtatccgctcatgagacaataaccctgataaatgcttcaataatattgaaaaaggaagagtatgagtattcaacatttccgtgtcgcccttattcccttttttgcggcattttgccttcctgtttttgctcacccagaaacgctggtgaaagtaaaagatgctgaagatcagttgggtgcacgagtgggttacatcgaactggatctcaacagcggtaagatccttgagagttttcgccccgaagaacgttttccaatgatgagcacttttaaagttctgctatgtggcgcggtattatcccgtattgacgccgggcaagagcaactcggtcgccgcatacactattctcagaatgacttggttgagtactcaccagtcacagaaaagcatcttacggatggcatgacagtaagagaattatgcagtgctgccataaccatgagtgataacactgcggccaacttacttctgacaacgatcggaggaccgaaggagctaaccgcttttttgcacaacatgggggatcatgtaactcgccttgatcgttgggaaccggagctgaatgaagccataccaaacgacgagcgtgacaccacgatgcctgtagcaatggcaacaacgttgcgcaaactattaactggcgaactacttactctagcttcccggcaacaattaatagactggatggaggcggataaagttgcaggaccacttctgcgctcggcccttccggctggctggtttattgctgataaatctggagccggtgagcgtggctctcgcggtatcattgcagcactggggccagatggtaagccctcccgtatcgtagttatctacacgacggggagtcaggcaactatggatgaacgaaatagacagatcgctgagataggtgcctcactgattaagcattggtaactgtcagaccaagtttactcatatatactttagattgatttaaaacttcatttttaatttaaaaggatctaggtgaagatcctttttgataatctcatgaccaaaatcccttaacgtgagttttcgttccactgagcgtcagaccccgtagaaaagatcaaaggatcttcttgagatcctttttttctgcgcgtaatctgctgcttgcaaacaaaaaaaccaccgctaccagcggtggtttgtttgccggatcaagagctaccaactctttttccgaaggtaactggcttcagcagagcgcagataccaaatactgttcttctagtgtagccgtagttaggccaccacttcaagaactctgtagcaccgcctacatacctcgctctgctaatcctgttaccagtggctgctgccagtggcgataagtcgtgtcttaccgggttggactcaagacgatagttaccggataaggcgcagcggtcgggctgaacggggggttcgtgcacacagcccagcttggagcgaacgacctacaccgaactgagatacctacagcgtgagctatgagaaagcgccacgcttcccgaagggagaaaggcggacaggtatccggtaagcggcagggtcggaacaggagagcgcacgagggagcttccagggggaaacgcctggtatctttatagtcctgtcgggtttcgccacctctgacttgagcgtcgatttttgtgatgctcgtcaggggggcggagcctatggaaaaacgccagcaacgcggcctttttacggttcctggccttttgctggccttttgctcacatgttctttcctgcgttatcccctgattctgtggataaccgtattaccgcctttgagtgagctgataccgctcgccgcagccgaacgaccgagcgcagcgagtcagtgagcgaggaagcggaagagcgcccaatacgcaaaccgcctctccccgcgcgttggccgattcattaatgcagctggcacgacaggtttcccgactggaaagcgggcagtgagcgcaacgcaattaatgtgagttagctcactcattaggcaccccaggctttacactttatgcttccggctcgtatgttgtgtggaattgtgagcggataacaatttcacacaggaaacagctatgaccatgattacgccaagcgcgcaattaaccctcactaaagggaacaaaagctggagctgcaagcttaatgtagtcttatgcaatactcttgtagtcttgcaacatggtaacgatgagttagcaacatgccttacaaggagagaaaaagcaccgtgcatgccgattggtggaagtaaggtggtacgatcgtgccttattaggaaggcaacagacgggtctgacatggattggacgaaccactgaattgccgcattgcagagatattgtatttaagtgcctagctcgatacataaacggctctctctggttagaccagatctgagcctgggagctctctggctaactagggaacccactgcttaagcctcaataaagcttgccttgagtgcttcaagtagtgtgtgcccgtctgttgtgtgactctggtaactagagatccctcagacccttttagtcagtgtggaaaatctctagcagtggcgcccgaacagggacttgaaagcgaaagggaaaccagaggagctctctcgacgcaggactcggcttgctgaagcgcgcacggcaagaggcgaggggcggcgactggtgagtacgccaaaaattttgactagcggaggctagaaggagagagatgggtgcgagagcgtcagtattaagcgggggagaattagatcgcgatgggaaaaaattcggttaaggccagggggaaagaaaaaatataaattaaaacatatagtatgggcaagcagggagctagaacgattcgcagttaatcctggcctgttagaaacatcagaaggctgtagacaaatactgggacagctacaaccatcccttcagacaggatcagaagaacttagatcattatataatacagtagcaaccctctattgtgtgcatcaaaggatagagataaaagacaccaaggaagctttagacaagatagaggaagagcaaaacaaaagtaagaccaccgcacagcaagcggccgctgatcttcagacctggaggaggagatatgagggacaattggagaagtgaattatataaatataaagtagtaaaaattgaaccattaggagtagcacccaccaaggcaaagagaagagtggtgcagagagaaaaaagagcagtgggaataggagctttgttccttgggttcttgggagcagcaggaagcactatgggcgcagcgtcaatgacgctgacggtacaggccagacaattattgtctggtatagtgcagcagcagaacaatttgctgagggctattgaggcgcaacagcatctgttgcaactcacagtctggggcatcaagcagctccaggcaagaatcctggctgtggaaagatacctaaaggatcaacagctcctggggatttggggttgctctggaaaactcatttgcaccactgctgtgccttggaatgctagttggagtaataaatctctggaacagatttggaatcacacgacctggatggagtgggacagagaaattaacaattacacaagcttaatacactccttaattgaagaatcgcaaaaccagcaagaaaagaatgaacaagaattattggaattagataaatgggcaagtttgtggaattggtttaacataacaaattggctgtggtatataaaattattcataatgatagtaggaggcttggtaggtttaagaatagtttttgctgtactttctatagtgaatagagttaggcagggatattcaccattatcgtttcagacccacctcccaaccccgaggggacccgacaggcccgaaggaatagaagaagaaggtggagagagagacagagacagatccattcgattagtgaacggatctcgacggtatcgatcacgagactagcctcgacacaaatggcagtattcatccacaattttaaaagaaaaggggggattggggggtacagtgcaggggaaagaatagtagacataatagcaacagacatacaaactaaagaattacaaaaacaaattacaaaaattcaaaattttcgggtttattacagggacagcagaaatccactttggctcgagaagcttgatatcggctccggtgcccgtcagtgggcagagcgcacatcgcccacagtccccgagaagttggggggaggggtcggcaattgaaccggtgcctagagaaggtggcgcggggtaaactgggaaagtgatgtcgtgtactggctccgcctttttcccgagggtgggggagaaccgtatataagtgcagtagtcgccgtgaacgttctttttcgcaacgggtttgccgccagaacacaggatccgccaccatggccttaccagtgaccgccttgctcctgccgctggccttgctgctccacgccgccaggccggatatccagatgacccagagcccgagcagcctgagcgcgagcgtgggtgatcgcgtgaccattacctgcagggcaagtcaggacattagtaaatatttaaattggtatcagcagaaaccgggtaaagcgccgaaactgttaatttatcatacatcaagattacactcaggcgtgccgtcgcgttttagcggctcgggttcgggcaccgattttaccctgaccatctcgagcttgcagccggaggacttcgccacctactattgccaacagggtaatacgcttccgtacacgttcggtcagggcaccaaagtggagatcaaaggtggcggtggctcgggcggtggtgggtcgggtggcggcggatctgaggtgcagctggtggagtctgggggaggcttggtacagcctggggggtccctgagactctcctgtgcagcctctggagtgtccctgcctgattatggcgtgtcctgggtccgccaggctccagggaaggggctggagtgggtttcagtgatctggggcagcgagacaacctactacaacagcgccctgaagtcccgattcaccatctccagagacaatgccaagaactcactgtatctgcaaatgaacagcctgagagccgaggacacggctgtgtattactgtgcgaagcactactactacggcggcagctacgctatggactactggggccaaggaaccctggtcaccgtgtcctcaaccacgacgccagcgccgcgaccaccaacaccggcgcccaccatcgcgtcgcagcccctgtccctgcgcccagaggcgtgccggccagcggcggggggcgcagtgcacacgagggggctggacttcgcctgtgatatctacatctgggcgcccttggccgggacttgtggggtccttctcctgtcactggttatcaccctttactgcaaacggggcagaaagaaactcctgtatatattcaaacaaccatttatgagaccagtacaaactactcaagaggaagatggctgtagctgccgatttccagaagaagaagaaggaggatgtgaactgagagtgaagttcagcaggagcgcagacgcccccgcgtacaagcagggccagaaccagctctataacgagctcaatctaggacgaagagaggagtacgatgttttggacaagaggcgtggccgggaccctgagatggggggaaagccgagaaggaagaaccctcaggaaggcctgtacaatgaactgcagaaagataagatggcggaggcctacagtgagattgggatgaaaggcgagcgccggaggggcaaggggcacgatggcctttaccagggtctcagtacagccaccaaggacacctacgacgcccttcacatgcaggccctgccccctcgctaatctagaggcgcgcc

SEQ ID NO: 11 - DNA, 7893 bp, Artificial Sequence
  synthesis
gtcgacactagtaatcaacctctggattacaaaatttgtgaaagattgactggtattcttaactatgttgctccttttacgctatgtggatacgctgctttaatgcctttgtatcatgctattgcttcccgtatggctttcattttctcctccttgtataaatcctggttgctgtctctttatgaggagttgtggcccgttgtcaggcaacgtggcgtggtgtgcactgtgtttgctgacgcaacccccactggttggggcattgccaccacctgtcagctcctttccgggactttcgctttccccctccctattgccacggcggaactcatcgccgcctgccttgcccgctgctggacaggggctcggctgttgggcactgacaattccgtggtgttgtcggggaagctgacgtcctttccatggctgctcgcctgtgttgccacctggattctgcgcgggacgtccttctgctacgtcccttcggccctcaatccagcggaccttccttcccgcggcctgctgccggctctgcggcctcttccgcgtcttcgccttcgccctcagacgagtcggatctccctttgggccgcctccccgcctgccgcggaattcgagctcggtacctttaagaccaatgacttacaaggcagctgtagatcttagccactttttaaaagaaaaggggggactggaagggctaattcactcccaacgaagacaagatctgctttttgcttgtactgagtctctctggttagaccagatctgagcctgggagctctctggctaactagggaacccactgcttaagcctcaataaagcttgccttgagtgcttcaagtagtgtgtgcccgtctgttgtgtgactctggtaactagagatccctcagacccttttagtcagtgtggaaaatctctagcagtagtagttcatgtcatcttattattcagtatttataacttgcaaagaaatgaatatcagagagtgagaggaacttgtttattgcagcttataatggttacaaataaagcaatagcatcacaaatttcacaaataaagcatttttttcactgcattctagttgtggtttgtccaaactcatcaatgtatcttatcatgtctggctctagctatcccgcccctaactccgcccatcccgcccctaactccgcccagttccgcccattctccgccccatggctgactaattttttttatttatgcagaggccgaggccgcctcggcctctgagctattccagaagtagtgaggaggcttttttggaggcctagggacgtacccaattcgccctatagtgagtcgtattacgcgcgctcactggccgtcgttttacaacgtcgtgactgggaaaaccctggcgttacccaacttaatcgccttgcagcacatccccctttcgccagctggcgtaatagcgaagaggcccgcaccgatcgcccttcccaacagttgcgcagcctgaatggcgaatgggacgcgccctgtagcggcgcattaagcgcggcgggtgtggtggttacgcgcagcgtgaccgctacacttgccagcgccctagcgcccgctcctttcgctttcttcccttcctttctcgccacgttcgccggctttccccgtcaagctctaaatcgggggctccctttagggttccgatttagtgctttacggcacctcgaccccaaaaaacttgattagggtgatggttcacgtagtgggccatcgccctgatagacggtttttcgccctttgacgttggagtccacgttctttaatagtggactcttgttccaaactggaacaacactcaaccctatctcggtctattcttttgatttataagggattttgccgatttcggcctattggttaaaaaatgagctgatttaacaaaaatttaacgcgaattttaacaaaatattaacgcttacaatttaggtggcacttttcggggaaatgtgcgcggaacccctatttgtttatttttctaaatacattcaaatatgtatccgctcatgagacaataaccctgataaatgcttcaataatattgaaaaaggaagagtatgagtattcaacatttccgtgtcgcccttattcccttttttgcggcattttgccttcctgtttttgctcacccagaaacgctggtgaaagtaaaagatgctgaagatcagttgggtgcacgagtgggttacatcgaactggatctcaacagcggtaagatccttgagagttttcgccccgaagaacgttttccaatgatgagcacttttaaagttctgctatgtggcgcggtattatcccgtattgacgccgggcaagagcaactcggtcgccgcatacactattctcagaatgacttggttgagtactcaccagtcacagaaaagcatcttacggatggcatgacagtaagagaattatgcagtgctgccataaccatgagtgataacactgcggccaacttacttctgacaacgatcggaggaccgaaggagctaaccgcttttttgcacaacatgggggatcatgtaactcgccttgatcgttgggaaccggagctgaatgaagccataccaaacgacgagcgtgacaccacgatgcctgtagcaatggcaacaacgttgcgcaaactattaactggcgaactacttactctagcttcccggcaacaattaatagactggatggaggcggataaagttgcaggaccacttctgcgctcggcccttccggctggctggtttattgctgataaatctggagccggtgagcgtggctctcgcggtatcattgcagcactggggccagatggtaagccctcccgtatcgtagttatctacacgacggggagtcaggcaactatggatgaacgaaatagacagatcgctgagataggtgcctcactgattaagcattggtaactgtcagaccaagtttactcatatatactttagattgatttaaaacttcatttttaatttaaaaggatctaggtgaagatcctttttgataatctcatgaccaaaatcccttaacgtgagttttcgttccactgagcgtcagaccccgtagaaaagatcaaaggatcttcttgagatcctttttttctgcgcgtaatctgctgcttgcaaacaaaaaaaccaccgctaccagcggtggtttgtttgccggatcaagagctaccaactctttttccgaaggtaactggcttcagcagagcgcagataccaaatactgttcttctagtgtagccgtagttaggccaccacttcaagaactctgtagcaccgcctacatacctcgctctgctaatcctgttaccagtggctgctgccagtggcgataagtcgtgtcttaccgggttggactcaagacgatagttaccggataaggcgcagcggtcgggctgaacggggggttcgtgcacacagcccagcttggagcgaacgacctacaccgaactgagatacctacagcgtgagctatgagaaagcgccacgcttcccgaagggagaaaggcggacaggtatccggtaagcggcagggtcggaacaggagagcgcacgagggagcttccagggggaaacgcctggtatctttatagtcctgtcgggtttcgccacctctgacttgagcgtcgatttttgtgatgctcgtcaggggggcggagcctatggaaaaacgccagcaacgcggcctttttacggttcctggccttttgctggccttttgctcacatgttctttcctgcgttatcccctgattctgtggataaccgtattaccgcctttgagtgagctgataccgctcgccgcagccgaacgaccgagcgcagcgagtcagtgagcgaggaagcggaagagcgcccaatacgcaaaccgcctctccccgcgcgttggccgattcattaatgcagctggcacgacaggtttcccgactggaaagcgggcagtgagcgcaacgcaattaatgtgagttagctcactcattaggcaccccaggctttacactttatgcttccggctcgtatgttgtgtggaattgtgagcggataacaatttcacacaggaaacagctatgaccatgattacgccaagcgcgcaattaaccctcactaaagggaacaaaagctggagctgcaagcttaatgtagtcttatgcaatactcttgtagtcttgcaacatggtaacgatgagttagcaacatgccttacaaggagagaaaaagcaccgtgcatgccgattggtggaagtaaggtggtacgatcgtgccttattaggaaggcaacagacgggtctgacatggattggacgaaccactgaattgccgcattgcagagatattgtatttaagtgcctagctcgatacataaacggctctctctggttagaccagatctgagcctgggagctctctggctaactagggaacccactgcttaagcctcaataaagcttgccttgagtgcttcaagtagtgtgtgcccgtctgttgtgtgactctggtaactagagatccctcagacccttttagtcagtgtggaaaatctctagcagtggcgcccgaacagggacttgaaagcgaaagggaaaccagaggagctctctcgacgcaggactcggcttgctgaagcgcgcacggcaagaggcgaggggcggcgactggtgagtacgccaaaaattttgactagcggaggctagaaggagagagatgggtgcgagagcgtcagtattaagcgggggagaattagatcgcgatgggaaaaaattcggttaaggccagggggaaagaaaaaatataaattaaaacatatagtatgggcaagcagggagctagaacgattcgcagttaatcctggcctgttagaaacatcagaaggctgtagacaaatactgggacagctacaaccatcccttcagacaggatcagaagaacttagatcattatataatacagtagcaaccctctattgtgtgcatcaaaggatagagataaaagacaccaaggaagctttagacaagatagaggaagagcaaaacaaaagtaagaccaccgcacagcaagcggccgctgatcttcagacctggaggaggagatatgagggacaattggagaagtgaattatataaatataaagtagtaaaaattgaaccattaggagtagcacccaccaaggcaaagagaagagtggtgcagagagaaaaaagagcagtgggaataggagctttgttccttgggttcttgggagcagcaggaagcactatgggcgcagcgtcaatgacgctgacggtacaggccagacaattattgtctggtatagtgcagcagcagaacaatttgctgagggctattgaggcgcaacagcatctgttgcaactcacagtctggggcatcaagcagctccaggcaagaatcctggctgtggaaagatacctaaaggatcaacagctcctggggatttggggttgctctggaaaactcatttgcaccactgctgtgccttggaatgctagttggagtaataaatctctggaacagatttggaatcacacgacctggatggagtgggacagagaaattaacaattacacaagcttaatacactccttaattgaagaatcgcaaaaccagcaagaaaagaatgaacaagaattattggaattagataaatgggcaagtttgtggaattggtttaacataacaaattggctgtggtatataaaattattcataatgatagtaggaggcttggtaggtttaagaatagtttttgctgtactttctatagtgaatagagttaggcagggatattcaccattatcgtttcagacccacctcccaaccccgaggggacccgacaggcccgaaggaatagaagaagaaggtggagagagagacagagacagatccattcgattagtgaacggatctcgacggtatcgatcacgagactagcctcgacacaaatggcagtattcatccacaattttaaaagaaaaggggggattggggggtacagtgcaggggaaagaatagtagacataatagcaacagacatacaaactaaagaattacaaaaacaaattacaaaaattcaaaattttcgggtttattacagggacagcagaaatccactttggctcgagaagcttgatatcggctccggtgcccgtcagtgggcagagcgcacatcgcccacagtccccgagaagttggggggaggggtcggcaattgaaccggtgcctagagaaggtggcgcggggtaaactgggaaagtgatgtcgtgtactggctccgcctttttcccgagggtgggggagaaccgtatataagtgcagtagtcgccgtgaacgttctttttcgcaacgggtttgccgccagaacacaggatccgccaccatggccttaccagtgaccgccttgctcctgccgctggccttgctgctccacgccgccaggccgcagatcgtgctgagccagagccccgccattctgagcgctagccccggcgagaaggtgaccatgacctgcagggccagcagcagcgtgagctacatccactggttccagcagaaacccggcagcagccccaagccctggatctacgccaccagcaacctggccagcggagtgcccgtgagatttagcggctccggcagcggcacctcctattccctgaccatctccagggtggaagccgaagacgccgccacctactactgccagcagtggaccagcaacccccctacctttggcggcggcaccaagctggagattaagggcggaggaagcggaggaggaagcggaggaggaagccaggtgcagctgcagcagcccggagccgaactggtgaagcccggagccagcgtgaagatgtcctgtaaggcctccggctacaccttcacctcctacaacatgcactgggtgaagcaaacccctggcagaggcctggagtggattggcgccatctaccccggcaacggcgacaccagctacaaccagaagttcaagggcaaggccaccctgaccgccgacaaaagcagcagcaccgcctatatgcagctgagctccctgacaagcgaggatagcgccgtgtactactgcgccagaagcacctactacggcggcgactggtacttcaacgtgtggggcgccggcaccacagtgacagtggcctccaccacgacgccagcgccgcgaccaccaacaccggcgcccaccatcgcgtcgcagcccctgtccctgcgcccagaggcgtgccggccagcggcggggggcgcagtgcacacgagggggctggacttcgcctgtgatatctacatctgggcgcccttggccgggacttgtggggtccttctcctgtcactggttatcaccctttactgcaaacggggcagaaagaaactcctgtatatattcaaacaaccatttatgagaccagtacaaactactcaagaggaagatggctgtagctgccgatttccagaagaagaagaaggaggatgtgaactgagagtgaagttcagcaggagcgcagacgcccccgcgtacaagcagggccagaaccagctctataacgagctcaatctaggacgaagagaggagtacgatgttttggacaagaggcgtggccgggaccctgagatggggggaaagccgagaaggaagaaccctcaggaaggcctgtacaatgaactgcagaaagataagatggcggaggcctacagtgagattgggatgaaaggcgagcgccggaggggcaaggggcacgatggcctttaccagggtctcagtacagccaccaaggacacctacgacgcccttcacatgcaggccctgccccctcgctaatctagaggcgcgcc

SEQ ID NO: 12 - DNA, 7902 bp, Artificial Sequence; identical to SEQ ID NO: 8
  synthesis

SEQ ID NO: 13 - DNA, 11052 bp, Artificial Sequence
  synthesis
caggtggcacttttcggggaaatgtgcgcggaacccctatttgtttatttttctaaatacattcaaatatgtatccgctcatgagacaataaccctgataaatgcttcaataatattgaaaaaggaagagtatgagtattcaacatttccgtgtcgcccttattcccttttttgcggcattttgccttcctgtttttgctcacccagaaacgctggtgaaagtaaaagatgctgaagatcagttgggtgcacgagtgggttacatcgaactggatctcaacagcggtaagatccttgagagttttcgccccgaagaacgttttccaatgatgagcacttttaaagttctgctatgtggcgcggtattatcccgtattgacgccgggcaagagcaactcggtcgccgcatacactattctcagaatgacttggttgagtactcaccagtcacagaaaagcatcttacggatggcatgacagtaagagaattatgcagtgctgccataaccatgagtgataacactgcggccaacttacttctgacaacgatcggaggaccgaaggagctaaccgcttttttgcacaacatgggggatcatgtaactcgccttgatcgttgggaaccggagctgaatgaagccataccaaacgacgagcgtgacaccacgatgcctgtagcaatggcaacaacgttgcgcaaactattaactggcgaactacttactctagcttcccggcaacaattaatagactggatggaggcggataaagttgcaggaccacttctgcgctcggcccttccggctggctggtttattgctgataaatctggagccggtgagcgtgggtctcgcggtatcattgcagcactggggccagatggtaagccctcccgtatcgtagttatctacacgacggggagtcaggcaactatggatgaacgaaatagacagatcgctgagataggtgcctcactgattaagcattggtaactgtcagaccaagtttactcatatatactttagattgatttaaaacttcatttttaatttaaaaggatctaggtgaagatcctttttgataatctcatgaccaaaatcccttaacgtgagttttcgttccactgagcgtcagaccccgtagaaaagatcaaaggatcttcttgagatcctttttttctgcgcgtaatctgctgcttgcaaacaaaaaaaccaccgctaccagcggtggtttgtttgccggatcaagagctaccaactctttttccgaaggtaactggcttcagcagagcgcagataccaaatactgtccttctagtgtagccgtagttaggccaccacttcaagaactctgtagcaccgcctacatacctcgctctgctaatcctgttaccagtggctgctgccagtggcgataagtcgtgtcttaccgggttggactcaagacgatagttaccggataaggcgcagcggtcgggctgaacggggggttcgtgcacacagcccagcttggagcgaacgacctacaccgaactgagatacctacagcgtgagctatgagaaagcgccacgcttcccgaagggagaaaggcggacaggtatccggtaagcggcagggtcggaacaggagagcgcacgagggagcttccagggggaaacgcctggtatctttatagtcctgtcgggtttcgccacctctgacttgagcgtcgatttttgtgatgctcgtcaggggggcggagcctatggaaaaacgccagcaacgcggcctttttacggttcctggccttttgctggccttttgctcacatgttctttcctgcgttatcccctgattctgtggataaccgtattaccgcctttgagtgagctgataccgctcgccgcagccgaacgaccgagcgcagcgagtcagtgagcgaggaagcggaagagcgcccaatacgcaaaccgcctctccccgcgcgttggccgattcattaatgcagctggcacgacaggtttcccgactggaaagcgggcagtgagcgcaacgcaattaatgtgagttagctcactcattaggcaccccaggctttacactttatgcttccggctcgtatgttgtgtggaattgtgagcggataacaatttcacacaggaaacagctatgaccatgattacgccaagcgcgcaattaaccctcactaaagggaacaaaagctggagctgcaagcttaatgtagtcttatgcaatactcttgtagtcttgcaacatggtaacgatgagttagcaacatgccttacaaggagagaaaaagcaccgtgcatgccgattggtggaagtaaggtggtacgatcgtgccttattaggaaggcaacagacgggtctgacatggattggacgaaccactgaattggaggcgtggcctgggcgggactggggagtggcgagccctcagatcctgcatataagcagctgctttttgcctgtactgggtctctctggttagaccagatctgagcctgggagctctctggctaactagggaacccactgcttaagcctcaataaagcttgccttgagtgcttcaagtagtgtgtgcccgtctgttgtgtgactctggtaactagagatccctcagacccttttagtcagtgtggaaaatctctagcagtggcgcccgaacagggacctgaaagcgaaagggaaaccagagctctctcgacgcaggactcggcttgctgaagcgcgcacggcaagaggcgaggggcggcgactggtgagtacgccaaaaattttgactagcggaggctagaaggagagagatgggtgcgagagcgtcagtattaagcgggggagaattagatcgcgatgggaaaaaattcggttaaggccagggggaaagaaaaaatataaattaaaacatatagtatgggcaagcagggagctagaacgattcgcagttaatcctggcctgttagaaacatcagaaggctgtagacaaatactgggacagctacaaccatcccttcagacaggatcagaagaacttagatcattatataatacagtagcaaccctctattgtgtgcatcaaaggatagagataaaagacaccaaggaagctttagacaagatagaggaagagcaaaacaaaagtaagaccaccgcacagcaagcggccgctgatcttcagacctggaggaggagatatgagggacaattggagaagtgaattatataaatataaagtagtaaaaattgaaccattaggagtagcacccaccaaggcaaagagaagagtggtgcagagagaaaaaagagcagtgggaataggagctttgttccttgggttcttgggagcagcaggaagcactatgggcgcagcctcaatgacgctgacggtacaggccagacaattattgtctggtatagtgcagcagcagaacaatttgctgagggctattgaggcgcaacagcatctgttgcaactcacagtctggggcatcaagcagctccaggcaagaatcctggctgtggaaagatacctaaaggatcaacagctcctggggatttggggttgctctggaaaactcatttgcaccactgctgtgccttggaatgctagttggagtaataaatctctggaacagattggaatcacacgacctggatggagtgggacagagaaattaacaattacacaagcttaatacactccttaattgaagaatcgcaaaaccagcaagaaaagaatgaacaagaattattggaattagataaatgggcaagtttgtggaattggtttaacataacaaattggctgtggtatataaaattattcataatgatagtaggaggcttggtaggtttaagaatagtttttgctgtactttctatagtgaatagagttaggcagggatattcaccattatcgtttcagacccacctcccaaccccgaggggacccgacaggcccgaaggaatagaagaagaaggtggagagagagacagagacagatccattcgattagtgaacggatctcgacggtatcgatcacgagactagcctcgacacaaatggcagtattcatccacaattttaaaagaaaaggggggattggggggtacagtgcaggggaaagaatagtagacataatagcaacagacatacaaactaaagaattacaaaaacaaattacaaaaattcaaaattttcgggtttattacagggacagcagaaatccactttggctcgagaagcttgatatcggctccggtgcccgtcagtgggcagagcgcacatcgcccacagtccccgagaagttggggggaggggtcggcaattgaaccggtgcctagagaaggtggcgcggggtaaactgggaaagtgatgtcgtgtactggctccgcctttttcccgagggtgggggagaaccgtatataagtgcagtagtcgccgtgaacgttctttttcgcaacgggtttgccgccagaacacagccaccatggcttcgtacccctgccatcaacacgcgtctgcgttcgaccaggctgcgcgttctcgcggccatagcaaccgacgtacggcgttgcgccctcgccggcagcaagaagccacggaagtccgcccggagcagaaaatgcccacgctactgcgggtttatatagacggtccccacgggatggggaaaaccaccaccacgcaactgctggtggccctgggttcgcgcgacgatatcgtctacgtacccgagccgatgacttactggcgggtgctgggggcttccgagacaatcgcgaacatctacaccacacaacaccgcctcgaccagggtgagatatcggccggggacgcggcggtggtaatgacaagcgcccagataacaatgggcatgccttatgccgtgaccgacgccgttctggctcctcatatcgggggggaggctgggagctcacatgccccgcccccggccctcaccctcatcttcgaccgccatcccatcgccgccctcctgtgctacccggccgcgcgataccttatgggcagcatgaccccccaggccgtgctggcgttcgtggccctcatcccgccgaccttgcccggcacaaacatcgtgttgggggcccttccggaggacagacacatcgaccgcctggccaaacgccagcgccccggcgagcggcttgacctggctatgctggccgcgattcgccgcgtttacgggctgcttgccaatacggtgcggtatctgcagggcggcgggtcgtggcgggaggattggggacagctttcggggacggccgtgccgccccagggtgccgagccccagagcaacgcgggcccacgaccccatatcggggacacgttatttaccctgtttcgggcccccgagttgctggcccccaacggcgacctgtataacgtgtttgcctgggccttggacgtcttggccaaacgcctccgtcccatgcacgtctttatcctggattacgaccaatcgcccgccggctgccgggacgccctgctgcaacttacctccgggatggtccagacccacgtcaccaccccaggctccataccgacgatctgcgacctggcgcgcacgtttgcccgggagatgggggaggctaactgacctctccctcccccccccctaacgttactggccgaagccgcttggaataaggccggtgtgcgtttgtctatatgttattttccaccatattgccgtcttttggcaatgtgagggcccggaaacctggccctgtcttcttgacgagcattcctaggggtctttcccctctcgccaaaggaatgcaaggtctgttgaatgtcgtgaaggaagcagttcctctggaagcttcttgaagacaaacaacgtctgtagcgaccctttgcaggcagcggaaccccccacctggcgacaggtgcctctgcggccaaaagccacgtgtataagatacacctgcaaaggcggcacaaccccagtgccacgttgtgagttggatagttgtggaaagagtcaaatggctctcctcaagcgtattcaacaaggggctgaaggatgcccagaaggtaccccattgtatgggatctgatctggggcctcggtacacatgctttacatgtgtttagtcgaggttaaaaaaacgtctaggccccccgaaccacggggacgtggttttcctttgaaaaacacgatgataatatggccacaaccatgtctagattagataaaagtaaagtgattaacagcgcattagagctgcttaatgaggtcggaatcgaaggtttaacaacccgtaaactcgcccagaagcttggtgtagagcagcctacactgtattggcatgtaaaaaataagcgggctttgctcgacgccttagccattgagatgttagataggcaccatactcacttttgccctttaaaaggggaaagctggcaagattttttacgcaataacgctaaaagttttagatgtgctttactaagtcatcgcaatggagcaaaagtacattcagatacacggcctacagaaaaacagtatgaaactctcgaaaatcaattagcctttttatgccaacaaggtttttcactagagaacgcgttatatgcactcagcgctgtggggcattttactttaggttgcgtattggaagatcaagagcatcaagtcgctaaagaagaaagggaaacacctactactgatagtatgccgccattattacgacaagctatcgaattatttgatcaccaaggtgcagagccagccttcttattcggccttgaattgatcatatgcggattagaaaaacaacttaaatgtgaaagtgggtccgcgtacagccgcgcgcgtacgaaaaacaattacgggtctaccatcgagggcctgctcgatctcccggacgacgacgcccccgaagaggcggggctggcggctccgcgcctgtcctttctccccgcgggacacacgcgcagactgtcgacggcccccccgaccgatgtcagcctgggggacgagctccacttagacggcgaggacgtggcgatggcgcatgccgacgcgctagacgatttcgatctggacatgttgggggacggggattccccgggtccgggatttaccccccacgactccgccccctacggcgctctggatatggccgacttcgagtttgagcagatgtttaccgatgcccttggaattgacgagtacggtgggtagctcgagtttaccactccctatcagtgatagagaaaagtgaaagtcgagtttaccactccctatcagtgatagagaaaagtgaaagtcgagtttaccactccctatcagtgatagagaaaagtgaaagtcgagtttaccactccctatcagtgatagagaaaagtgaaagtcgagtttaccactccctatcagtgatagagaaaagtgaaagtcgagtttaccactccctatcagtgatagagaaaagtgaaagtcgagtttaccactccctatcagtgatagagaaaagtgaaagtcgagctcggtacccgggtcgagtaggcgtgtacggtgggaggcctatataagcagagctcgtttagtgaaccgtcagatcgcctggagacgccatccacgctgttttgacctccatagaagacaccgggaccgatccagcctatgccgcgcgctccccgctgccgagccgtgcgctccctgctgcgcagccactaccgcgaggtgctgccgctggccacgttcgtgcggcgcctggggccccagggctggcggctggtgcagcgcggggacccggcggctttccgcgcgctggtggcccagtgcctggtgtgcgtgccctgggacgcacggccgccccccgccgccccctccttccgccaggtgtcctgcctgaaggagctggtggcccgagtgctgcagaggctgtgcgagcgcggcgcgaagaacgtgctggccttcggcttcgcgctgctggacggggcccgcgggggcccccccgaggccttcaccaccagcgtgcgcagctacctgcccaacacggtgaccgacgcactgcgggggagcggggcgtgggggctgctgctgcgccgcgtgggcgacgacgtgctggttcacctgctggcacgctgcgcgctctttgtgctggtggctcccagctgcgcctaccaggtgtgcgggccgccgctgtaccagctcggcgctgccactcaggcccggcccccgccacacgctagtggaccccgaaggcgtctgggatgcgaacgggcctggaaccatagcgtcagggaggccggggtccccctgggcctgccagccccgggtgcgaggaggcgcgggggcagtgccagccgaagtctgccgttgcccaagaggcccaggcgtggcgctgcccctgagccggagcggacgcccgttgggcaggggtcctgggcccacccgggcaggacgcgtggaccgagtgaccgtggtttctgtgtggtgtcacctgccagacccgccgaagaagccacctctttggagggtgcgctctctggcacgcgccactcccacccatccgtgggccgccagcaccacgcgggccccccatccacatcgcggccaccacgtccctgggacacgccttgtcccccggtgtacgccgagaccaagcacttcctctactcctcaggcgacaaggagcagctgcggccctccttcctactcagctctctgaggcccagcctgactggcgctcggaggctcgtggagaccatctttctgggttccaggccctggatgccagggactccccgcaggttgccccgcctgccccagcgctactggcaaatgcggcccctgtttctggagctgcttgggaaccacgcgcagtgcccctacggggtgctcctcaagacgcactgcccgctgcgagctgcggtcaccccagcagccggtgtctgtgcccgggagaagccccagggctctgtggcggcccccgaggaggaggacacagacccccgtcgcctggtgcagctgctccgccagcacagcagcccctggcaggtgtacggcttcgtgcgggcctgcctgcgccggctggtgcccccaggcctctggggctccaggcacaacgaacgccgcttcctcaggaacaccaagaagttcatctccctggggaagcatgccaagctctcgctgcaggagctgacgtggaagatgagcgtgcgggactgcgcttggctgcgcaggagcccaggggttggctgtgttccggccgcagagcaccgtctgcgtgaggagatcctggccaagttcctgcactggctgatgagtgtgtacgtcgtcgagctgctcaggtctttcttttatgtcacggagaccacgtttcaaaagaacaggctctttttctaccggaagagtgtctggagcaagttgcaaagcattggaatcagacagcacttgaagagggtgcagctgcgggagctgtcggaagcagaggtcaggcagcatcgggaagccaggcccgccctgctgacgtccagactccgcttcatccccaagcctgacgggctgcggccgattgtgaacatggactacgtcgtgggagccagaacgttccgcagagaaaagagggccgagcgtctcacctcgagggtgaaggcactgttcagcgtgctcaactacgagcgggcgcggcgccccggcctcctgggcgcctctgtgctgggcctggacgatatccacagggcctggcgcaccttcgtgctgcgtgtgcgggcccaggacccgccgcctgagctgtactttgtcaaggtggatgtgacgggcgcgtacgacaccatcccccaggacaggctcacggaggtcatcgccagcatcatcaaaccccagaacacgtactgcgtgcgtcggtatgccgtggtccagaaggccgcccatgggcacgtccgcaaggccttcaagagccacgtctctaccttgacagacctccagccgtacatgcgacagttcgtggctcacctgcaggagaccagcccgctgagggatgccgtcgtcatcgagcagagctcctccctgaatgaggccagcagtggcctcttcgacgtcttcctacgcttcatgtgccaccacgccgtgcgcatcaggggcaagtcctacgtccagtgccaggggatcccgcagggctccatcctctccacgctgctctgcagcctgtgctacggcgacatggagaacaagctgtttgcggggattcggcgggacgggctgctcctgcgtttggtggatgatttcttgttggtgacacctcacctcacccacgcgaaaaccttcctcaggaccctggtccgaggtgtccctgagtatggctgcgtggtgaacttgcggaagacagtggtgaacttccctgtagaagacgaggccctgggtggcacggcttttgttcagatgccggcccacggcctattcccctggtgcggcctgctgctggatacccggaccctggaggtgcagagcgactactccagctatgcccggacctccatcagagccagtctcaccttcaaccgcggcttcaaggctgggaggaacatgcgtcgcaaactctttggggtcttgcggctgaagtgtcacagcctgtttctggatttgcaggtgaacagcctccagacggtgtgcaccaacatctacaagatcctcctgctgcaggcgtacaggtttcacgcatgtgtgctgcagctcccatttcatcagcaagtttggaagaaccccacatttttcctgcgcgtcatctctgacacggcctccctctgctactccatcctgaaagccaagaacgcagggatgtcgctgggggccaagggcgccgccggccctctgccctccgaggccgtgcagtggctgtgccaccaagcattcctgctcaagctgactcgacaccgtgtcacctacgtgccactcctggggtcactcaggacagcccagacgcagctgagtcggaagctcccggggacgacgctgactgccctggaggccgcagccaacccggcactgccctcagacttcaagaccatcctggactga

SEQ ID NO: 14 - DNA, 9780 bp, Artificial Sequence
  synthesis
caggtggcacttttcggggaaatgtgcgcggaacccctatttgtttatttttctaaatacattcaaatatgtatccgctcatgagacaataaccctgataaatgcttcaataatattgaaaaaggaagagtatgagtattcaacatttccgtgtcgcccttattcccttttttgcggcattttgccttcctgtttttgctcacccagaaacgctggtgaaagtaaaagatgctgaagatcagttgggtgcacgagtgggttacatcgaactggatctcaacagcggtaagatccttgagagttttcgccccgaagaacgttttccaatgatgagcacttttaaagttctgctatgtggcgcggtattatcccgtattgacgccgggcaagagcaactcggtcgccgcatacactattctcagaatgacttggttgagtactcaccagtcacagaaaagcatcttacggatggcatgacagtaagagaattatgcagtgctgccataaccatgagtgataacactgcggccaacttacttctgacaacgatcggaggaccgaaggagctaaccgcttttttgcacaacatgggggatcatgtaactcgccttgatcgttgggaaccggagctgaatgaagccataccaaacgacgagcgtgacaccacgatgcctgtagcaatggcaacaacgttgcgcaaactattaactggcgaactacttactctagcttcccggcaacaattaatagactggatggaggcggataaagttgcaggaccacttctgcgctcggcccttccggctggctggtttattgctgataaatctggagccggtgagcgtgggtctcgcggtatcattgcagcactggggccagatggtaagccctcccgtatcgtagttatctacacgacggggagtcaggcaactatggatgaacgaaatagacagatcgctgagataggtgcctcactgattaagcattggtaactgtcagaccaagtttactcatatatactttagattgatttaaaacttcatttttaatttaaaaggatctaggtgaagatcctttttgataatctcatgaccaaaatcccttaacgtgagttttcgttccactgagcgtcagaccccgtagaaaagatcaaaggatcttcttgagatcctttttttctgcgcgtaatctgctgcttgcaaacaaaaaaaccaccgctaccagcggtggtttgtttgccggatcaagagctaccaactctttttccgaaggtaactggcttcagcagagcgcagataccaaatactgtccttctagtgtagccgtagttaggccaccacttcaagaactctgtagcaccgcctacatacctcgctctgctaatcctgttaccagtggctgctgccagtggcgataagtcgtgtcttaccgggttggactcaagacgatagttaccggataaggcgcagcggtcgggctgaacggggggttcgtgcacacagcccagcttggagcgaacgacctacaccgaactgagatacctacagcgtgagctatgagaaagcgccacgcttcccgaagggagaaaggcggacaggtatccggtaagcggcagggtcggaacaggagagcgcacgagggagcttccagggggaaacgcctggtatctttatagtcctgtcgggtttcgccacctctgacttgagcgtcgatttttgtgatgctcgtcaggggggcggagcctatggaaaaacgccagcaacgcggcctttttacggttcctggccttttgctggccttttgctcacatgttctttcctgcgttatcccctgattctgtggataaccgtattaccgcctttgagtgagctgataccgctcgccgcagccgaacgaccgagcgcagcgagtcagtgagcgaggaagcggaagagcgcccaatacgcaaaccgcctctccccgcgcgttggccgattcattaatgcagctggcacgacaggtttcccgactggaaagcgggcagtgagcgcaacgcaattaatgtgagttagctcactcattaggcaccccaggctttacactttatgcttccggctcgtatgttgtgtggaattgtgagcggataacaatttcacacaggaaacagctatgaccatgattacgccaagcgcgcaattaaccctcactaaagggaacaaaagctggagctgcaagcttaatgtagtcttatgcaatactcttgtagtcttgcaacatggtaacgatgagttagcaacatgccttacaaggagagaaaaagcaccgtgcatgccgattggtggaagtaaggtggtacgatcgtgccttattaggaaggcaacagacgggtctgacatggattggacgaaccactgaattggaggcgtggcctgggcgggactggggagtggcgagccctcagatcctgcatataagcagctgctttttgcctgtactgggtctctctggttagaccagatctgagcctgggagctctctggctaactagggaacccactgcttaagcctcaataaagcttgccttgagtgcttcaagtagtgtgtgcccgtctgttgtgtgactctggtaactagagatccctcagacccttttagtcagtgtggaaaatctctagcagtggcgcccgaacagggacctgaaagcgaaagggaaaccagagctctctcgacgcaggactcggcttgctgaagcgcgcacggcaagaggcgaggggcggcgactggtgagtacgccaaaaattttgactagcggaggctagaaggagagagatgggtgcgagagcgtcagtattaagcgggggagaattagatcgcgatgggaaaaaattcggttaaggccagggggaaagaaaaaatataaattaaaacatatagtatgggcaagcagggagctagaacgattcgcagttaatcctggcctgttagaaacatcagaaggctgtagacaaatactgggacagctacaaccatcccttcagacaggatcagaagaacttagatcattatataatacagtagcaaccctctattgtgtgcatcaaaggatagagataaaagacaccaaggaagctttagacaagatagaggaagagcaaaacaaaagtaagaccaccgcacagcaagcggccgctgatcttcagacctggaggaggagatatgagggacaattggagaagtgaattatataaatataaagtagtaaaaattgaaccattaggagtagcacccaccaaggcaaagagaagagtggtgcagagagaaaaaagagcagtgggaataggagctttgttccttgggttcttgggagcagcaggaagcactatgggcgcagcctcaatgacgctgacggtacaggccagacaattattgtctggtatagtgcagcagcagaacaatttgctgagggctattgaggcgcaacagcatctgttgcaactcacagtctggggcatcaagcagctccaggcaagaatcctggctgtggaaagatacctaaaggatcaacagctcctggggatttggggttgctctggaaaactcatttgcaccactgctgtgccttggaatgctagttggagtaataaatctctggaacagattggaatcacacgacctggatggagtgggacagagaaattaacaattacacaagcttaatacactccttaattgaagaatcgcaaaaccagcaagaaaagaatgaacaagaattattggaattagataaatgggcaagtttgtggaattggtttaacataacaaattggctgtggtatataaaattattcataatgatagtaggaggcttggtaggtttaagaatagtttttgctgtactttctatagtgaatagagttaggcagggatattcaccattatcgtttcagacccacctcccaaccccgaggggacccgacaggcccgaaggaatagaagaagaaggtggagagagagacagagacagatccattcgattagtgaacggatctcgacggtatcgatcacgagactagcctcgacacaaatggcagtattcatccacaattttaaaagaaaaggggggattggggggtacagtgcaggggaaagaatagtagacataatagcaacagacatacaaactaaagaattacaaaaacaaattacaaaaattcaaaattttcgggtttattacagggacagcagaaatccactttggctcgagaagcttgatatcggctccggtgcccgtcagtgggcagagcgcacatcgcccacagtccccgagaagttggggggaggggtcggcaattgaaccggtgcctagagaaggtggcgcggggtaaactgggaaagtgatgtcgtgtactggctccgcctttttcccgagggtgggggagaaccgtatataagtgcagtagtcgccgtgaacgttctttttcgcaacgggtttgccgccagaacacagccaccatggcttcgtacccctgccatcaacacgcgtctgcgttcgaccaggctgcgcgttctcgcggccatagcaaccgacgtacggcgttgcgccctcgccggcagcaagaagccacggaagtccgcccggagcagaaaatgcccacgctactgcgggtttatatagacggtccccacgggatggggaaaaccaccaccacgcaactgctggtggccctgggttcgcgcgacgatatcgtctacgtacccgagccgatgacttactggcgggtgctgggggcttccgagacaatcgcgaacatctacaccacacaacaccgcctcgaccagggtgagatatcggccggggacgcggcggtggtaatgacaagcgcccagataacaatgggcatgccttatgccgtgaccgacgccgttctggctcctcatatcgggggggaggctgggagctcacatgccccgcccccggccctcaccctcatcttcgaccgccatcccatcgccgccctcctgtgctacccggccgcgcgataccttatgggcagcatgaccccccaggccgtgctggcgttcgtggccctcatcccgccgaccttgcccggcacaaacatcgtgttgggggcccttccggaggacagacacatcgaccgcctggccaaacgccagcgccccggcgagcggcttgacctggctatgctggccgcgattcgccgcgtttacgggctgcttgccaatacggtgcggtatctgcagggcggcgggtcgtggcgggaggattggggacagctttcggggacggccgtgccgccccagggtgccgagccccagagcaacgcgggcccacgaccccatatcggggacacgttatttaccctgtttcgggcccccgagttgctggcccccaacggcgacctgtataacgtgtttgcctgggccttggacgtcttggccaaacgcctccgtcccatgcacgtctttatcctggattacgaccaatcgcccgccggctgccgggacgccctgctgcaacttacctccgggatggtccagacccacgtcaccaccccaggctccataccgacgatctgcgacctggcgcgcacgtttgcccgggagatgggggaggctaactgacctctccctcccccccccctaacgttactggccgaagccgcttggaataaggccggtgtgcgtttgtctatatgttattttccaccatattgccgtcttttggcaatgtgagggcccggaaacctggccctgtcttcttgacgagcattcctaggggtctttcccctctcgccaaaggaatgcaaggtctgttgaatgtcgtgaaggaagcagttcctctggaagcttcttgaagacaaacaacgtctgtagcgaccctttgcaggcagcggaaccccccacctggcgacaggtgcctctgcggccaaaagccacgtgtataagatacacctgcaaaggcggcacaaccccagtgccacgttgtgagttggatagttgtggaaagagtcaaatggctctcctcaagcgtattcaacaaggggctgaaggatgcccagaaggtaccccattgtatgggatctgatctggggcctcggtacacatgctttacatgtgtttagtcgaggttaaaaaaacgtctaggccccccgaaccacggggacgtggttttcctttgaaaaacacgatgataatatggccacaaccatgtctagattagataaaagtaaagtgattaacagcgcattagagctgcttaatgaggtcggaatcgaaggtttaacaacccgtaaactcgcccagaagcttggtgtagagcagcctacactgtattggcatgtaaaaaataagcgggctttgctcgacgccttagccattgagatgttagataggcaccatactcacttttgccctttaaaaggggaaagctggcaagattttttacgcaataacgctaaaagttttagatgtgctttactaagtcatcgcaatggagcaaaagtacattcagatacacggcctacagaaaaacagtatgaaactctcgaaaatcaattagcctttttatgccaacaaggtttttcactagagaacgcgttatatgcactcagcgctgtggggcattttactttaggttgcgtattggaagatcaagagcatcaagtcgctaaagaagaaagggaaacacctactactgatagtatgccgccattattacgacaagctatcgaattatttgatcaccaaggtgcagagccagccttcttattcggccttgaattgatcatatgcggattagaaaaacaacttaaatgtgaaagtgggtccgcgtacagccgcgcgcgtacgaaaaacaattacgggtctaccatcgagggcctgctcgatctcccggacgacgacgcccccgaagaggcggggctggcggctccgcgcctgtcctttctccccgcgggacacacgcgcagactgtcgacggcccccccgaccgatgtcagcctgggggacgagctccacttagacggcgaggacgtggcgatggcgcatgccgacgcgctagacgatttcgatctggacatgttgggggacggggattccccgggtccgggatttaccccccacgactccgccccctacggcgctctggatatggccgacttcgagtttgagcagatgtttaccgatgcccttggaattgacgagtacggtgggtagctcgagtttaccactccctatcagtgatagagaaaagtgaaagtcgagtttaccactccctatcagtgatagagaaaagtgaaagtcgagtttaccactccctatcagtgatagagaaaagtgaaagtcgagtttaccactccctatcagtgatagagaaaagtgaaagtcgagtttaccactccctatcagtgatagagaaaagtgaaagtcgagtttaccactccctatcagtgatagagaaaagtgaaagtcgagtttaccactccctatcagtgatagagaaaagtgaaagtcgagctcggtacccgggtcgagtaggcgtgtacggtgggaggcctatataagcagagctcgtttagtgaaccgtcagatcgcctggagacgccatccacgctgttttgacctccatagaagacaccgggaccgatccagcctatggataaagttttaaacagagaggaatctttgcagctaatggaccttctaggtcttgaaaggagtgcctgggggaatattcctctgatgagaaaggcatatttaaaaaaatgcaaggagtttcatcctgataaaggaggagatgaagaaaaaatgaagaaaatgaatactctgtacaagaaaatggaagatggagtaaaatatgctcatcaacctgactttggaggcttctgggatgcaactgagattccaacctatggaactgatgaatgggagcagtggtggaatgcctttaatgaggaaaacctgttttgctcagaagaaatgccatctagtgatgatgaggctactgctgactctcaacattctactcctccaaaaaagaagagaaaggtagaagaccccaaggactttccttcagaattgctaagttttttgagtcatgctgtgtttagtaatagaactcttgcttgctttgctatttacaccacaaaggaaaaagctgcactgctatacaagaaaattatggaaaaatattctgtaacctttataagtaggcataacagttataatcataacatactgttttttcttactccacacaggcatagagtgtctgctattaataactatgctcaaaaattgtgtacctttagctttttaatttgtaaaggggttaataaggaatatttgatgtatagtgccttgactagagatccattttctgttattgaggaaagtttgccaggtgggttaaaggagcatgattttaatccagaagaagcagaggaaactaaacaagtgtcctggaagcttgtaacagagtatgcaatggaaacaaaatgtgatgatgtgttgttattgcttgggatgtacttggaatttcagtacagttttgaaatgtgtttaaaatgtattaaaaaagaacagcccagccactataagtaccatgaaaagcattatgcaaatgctgctatatttgctgacagcaaaaaccaaaaaaccatatgccaacaggctgttgatactgttttagctaaaaagcgggttgatagcctacaattaactagagaacaaatgttaacaaacagatttaatgatcttttggataggatggatataatgtttggttctacaggctctgctgacatagaagaatggatggctggagttgcttggctacactgtttgttgcccaaaatggattcagtggtgtatgactttttaaaatgcatggtgtacaacattcctaaaaaaagatactggctgtttaaaggaccaattgatagtggtaaaactacattagcagctgctttgcttgaattatgtggggggaaagctttaaatgttaatttgcccttggacaggctgaactttgagctaggagtagctattgaccagtttttagtagtttttgaggatgtaaagggcactggaggggagtccagagatttgccttcaggtcagggaattaataacctggacaatttaagggattatttggatggcagtgttaaggtaaacttagaaaagaaacacctaaataaaagaactcaaatatttccccctggaatagtcaccatgaatgagtacagtgtgcctaaaacactgcaggccagatttgtaaaacaaatagattttaggcccaaagattatttaaagcattgcctggaacgcagtgagtttttgttagaaaagagaataattcaaagtggcattgctttgcttcttatgttaatttggtacagacctgtggctgagtttgctcaaagtattcagagcagaattgtggagtggaaagagagattggacaaagagtttagtttgtcagtgtatcaaaaaatgaagtttaatgtggctatgggaattggagttttagattggctaagaaacagtgatgatgatgatgaagacagccaggaaaatgctgataaaaatgaagatggtggggagaagaacatggaagactcagggcatgaaacaggcattgattcacagtcccaaggctcatttcaggcccctcagtcctcacagtctgttcatgatcataatcagccataccacatttgtagaggttttacttgctttaaaaaacctcccacacctccccctgaacctgaaacataa

SEQ ID NO: 15 - DNA, 9840 bp, Artificial Sequence
  synthesis
gtcgacactagtaatcaacctctggattacaaaatttgtgaaagattgactggtattcttaactatgttgctccttttacgctatgtggatacgctgctttaatgcctttgtatcatgctattgcttcccgtatggctttcattttctcctccttgtataaatcctggttgctgtctctttatgaggagttgtggcccgttgtcaggcaacgtggcgtggtgtgcactgtgtttgctgacgcaacccccactggttggggcattgccaccacctgtcagctcctttccgggactttcgctttccccctccctattgccacggcggaactcatcgccgcctgccttgcccgctgctggacaggggctcggctgttgggcactgacaattccgtggtgttgtcggggaagctgacgtcctttccatggctgctcgcctgtgttgccacctggattctgcgcgggacgtccttctgctacgtcccttcggccctcaatccagcggaccttccttcccgcggcctgctgccggctctgcggcctcttccgcgtcttcgccttcgccctcagacgagtcggatctccctttgggccgcctccccgcctgccgcggaattcgagctcggtacctttaagaccaatgacttacaaggcagctgtagatcttagccactttttaaaagaaaaggggggactggaagggctaattcactcccaacgaagacaagatctgctttttgcttgtactgagtctctctggttagaccagatctgagcctgggagctctctggctaactagggaacccactgcttaagcctcaataaagcttgccttgagtgcttcaagtagtgtgtgcccgtctgttgtgtgactctggtaactagagatccctcagacccttttagtcagtgtggaaaatctctagcagtagtagttcatgtcatcttattattcagtatttataacttgcaaagaaatgaatatcagagagtgagaggaacttgtttattgcagcttataatggttacaaataaagcaatagcatcacaaatttcacaaataaagcatttttttcactgcattctagttgtggtttgtccaaactcatcaatgtatcttatcatgtctggctctagctatcccgcccctaactccgcccatcccgcccctaactccgcccagttccgcccattctccgccccatggctgactaattttttttatttatgcagaggccgaggccgcctcggcctctgagctattccagaagtagtgaggaggcttttttggaggcctagggacgtacccaattcgccctatagtgagtcgtattacgcgcgctcactggccgtcgttttacaacgtcgtgactgggaaaaccctggcgttacccaacttaatcgccttgcagcacatccccctttcgccagctggcgtaatagcgaagaggcccgcaccgatcgcccttcccaacagttgcgcagcctgaatggcgaatgggacgcgccctgtagcggcgcattaagcgcggcgggtgtggtggttacgcgcagcgtgaccgctacacttgccagcgccctagcgcccgctcctttcgctttcttcccttcctttctcgccacgttcgccggctttccccgtcaagctctaaatcgggggctccctttagggttccgatttagtgctttacggcacctcgaccccaaaaaacttgattagggtgatggttcacgtagtgggccatcgccctgatagacggtttttcgccctttgacgttggagtccacgttctttaatagtggactcttgttccaaactggaacaacactcaaccctatctcggtctattcttttgatttataagggattttgccgatttcggcctattggttaaaaaatgagctgatttaacaaaaatttaacgcgaattttaacaaaatattaacgcttacaatttaggtggcacttttcggggaaatgtgcgcggaacccctatttgtttatttttctaaatacattcaaatatgtatccgctcatgagacaataaccctgataaatgcttcaataatattgaaaaaggaagagtatgagtattcaacatttccgtgtcgcccttattcccttttttgcggcattttgccttcctgtttttgctcacccagaaacgctggtgaaagtaaaagatgctgaagatcagttgggtgcacgagtgggttacatcgaactggatctcaacagcggtaagatccttgagagttttcgccccgaagaacgttttccaatgatgagcacttttaaagttctgctatgtggcgcggtattatcccgtattgacgccgggcaagagcaactcggtcgccgcatacactattctcagaatgacttggttgagtactcaccagtcacagaaaagcatcttacggatggcatgacagtaagagaattatgcagtgctgccataaccatgagtgataacactgcggccaacttacttctgacaacgatcggaggaccgaaggagctaaccgcttttttgcacaacatgggggatcatgtaactcgccttgatcgttgggaaccggagctgaatgaagccataccaaacgacgagcgtgacaccacgatgcctgtagcaatggcaacaacgttgcgcaaactattaactggcgaactacttactctagcttcccggcaacaattaatagactggatggaggcggataaagttgcaggaccacttctgcgctcggcccttccggctggctggtttattgctgataaatctggagccggtgagcgtggctctcgcggtatcattgcagcactggggccagatggtaagccctcccgtatcgtagttatctacacgacggggagtcaggcaactatggatgaacgaaatagacagatcgctgagataggtgcctcactgattaagcattggtaactgtcagaccaagtttactcatatatactttagattgatttaaaacttcatttttaatttaaaaggatctaggtgaagatcctttttgataatctcatgaccaaaatcccttaacgtgagttttcgttccactgagcgtcagaccccgtagaaaagatcaaaggatcttcttgagatcctttttttctgcgcgtaatctgctgcttgcaaacaaaaaaaccaccgctaccagcggtggtttgtttgccggatcaagagctaccaactctttttccgaaggtaactggcttcagcagagcgcagataccaaatactgttcttctagtgtagccgtagttaggccaccacttcaagaactctgtagcaccgcctacatacctcgctctgctaatcctgttaccagtggctgctgccagtggcgataagtcgtgtcttaccgggttggactcaagacgatagttaccggataaggcgcagcggtcgggctgaacggggggttcgtgcacacagcccagcttggagcgaacgacctacaccgaactgagatacctacagcgtgagctatgagaaagcgccacgcttcccgaagggagaaaggcggacaggtatccggtaagcggcagggtcggaacaggagagcgcacgagggagcttccagggggaaacgcctggtatctttatagtcctgtcgggtttcgccacctctgacttgagcgtcgatttttgtgatgctcgtcaggggggcggagcctatggaaaaacgccagcaacgcggcctttttacggttcctggccttttgctggccttttgctcacatgttctttcctgcgttatcccctgattctgtggataaccgtattaccgcctttgagtgagctgataccgctcgccgcagccgaacgaccgagcgcagcgagtcagtgagcgaggaagcggaagagcgcccaatacgcaaaccgcctctccccgcgcgttggccgattcattaatgcagctggcacgacaggtttcccgactggaaagcgggcagtgagcgcaacgcaattaatgtgagttagctcactcattaggcaccccaggctttacactttatgcttccggctcgtatgttgtgtggaattgtgagcggataacaatttcacacaggaaacagctatgaccatgattacgccaagcgcgcaattaaccctcactaaagggaacaaaagctggagctgcaagcttaatgtagtcttatgcaatactcttgtagtcttgcaacatggtaacgatgagttagcaacatgccttacaaggagagaaaaagcaccgtgcatgccgattggtggaagtaaggtggtacgatcgtgccttattaggaaggcaacagacgggtctgacatggattggacgaaccactgaattgccgcattgcagagatattgtatttaagtgcctagctcgatacataaacggctctctctggttagaccagatctgagcctgggagctctctggctaactagggaacccactgcttaagcctcaataaagcttgccttgagtgcttcaagtagtgtgtgcccgtctgttgtgtgactctggtaactagagatccctcagacccttttagtcagtgtggaaaatctctagcagtggcgcccgaacagggacttgaaagcgaaagggaaaccagaggagctctctcgacgcaggactcggcttgctgaagcgcgcacggcaagaggcgaggggcggcgactggtgagtacgccaaaaattttgactagcggaggctagaaggagagagatgggtgcgagagcgtcagtattaagcgggggagaattagatcgcgatgggaaaaaattcggttaaggccagggggaaagaaaaaatataaattaaaacatatagtatgggcaagcagggagctagaacgattcgcagttaatcctggcctgttagaaacatcagaaggctgtagacaaatactgggacagctacaaccatcccttcagacaggatcagaagaacttagatcattatataatacagtagcaaccctctattgtgtgcatcaaaggatagagataaaagacaccaaggaagctttagacaagatagaggaagagcaaaacaaaagtaagaccaccgcacagcaagcggccgctgatcttcagacctggaggaggagatatgagggacaattggagaagtgaattatataaatataaagtagtaaaaattgaaccattaggagtagcacccaccaaggcaaagagaagagtggtgcagagagaaaaaagagcagtgggaataggagctttgttccttgggttcttgggagcagcaggaagcactatgggcgcagcgtcaatgacgctgacggtacaggccagacaattattgtctggtatagtgcagcagcagaacaatttgctgagggctattgaggcgcaacagcatctgttgcaactcacagtctggggcatcaagcagctccaggcaagaatcctggctgtggaaagatacctaaaggatcaacagctcctggggatttggggttgctctggaaaactcatttgcaccactgctgtgccttggaatgctagttggagtaataaatctctggaacagatttggaatcacacgacctggatggagtgggacagagaaattaacaattacacaagcttaatacactccttaattgaagaatcgcaaaaccagcaagaaaagaatgaacaagaattattggaattagataaatgggcaagtttgtggaattggtttaacataacaaattggctgtggtatataaaattattcataatgatagtaggaggcttggtaggtttaagaatagtttttgctgtactttctatagtgaatagagttaggcagggatattcaccattatcgtttcagacccacctcccaaccccgaggggacccgacaggcccgaaggaatagaagaagaaggtggagagagagacagagacagatccattcgattagtgaacggatctcgacggtatcgatcacgagactagcctcgacacaaatggcagtattcatccacaattttaaaagaaaaggggggattggggggtacagtgcaggggaaagaatagtagacataatagcaacagacatacaaactaaagaattacaaaaacaaattacaaaaattcaaaattttcgggtttattacagggacagcagaaatccactttggctcgagaagcttgatatcggctccggtgcccgtcagtgggcagagcgcacatcgcccacagtccccgagaagttggggggaggggtcggcaattgaaccggtgcctagagaaggtggcgcggggtaaactgggaaagtgatgtcgtgtactggctccgcctttttcccgagggtgggggagaaccgtatataagtgcagtagtcgccgtgaacgttctttttcgcaacgggtttgccgccagaacacaggatccgccaccatgccgcgcgctccccgctgccgagccgtgcgctccctgctgcgcagccactaccgcgaggtgctgccgctggccacgttcgtgcggcgcctggggccccagggctggcggctggtgcagcgcggggacccggcggctttccgcgcgctggtggcccagtgcctggtgtgcgtgccctgggacgcacggccgccccccgccgccccctccttccgccaggtgtcctgcctgaaggagctggtggcccgagtgctgcagaggctgtgcgagcgcggcgcgaagaacgtgctggccttcggcttcgcgctgctggacggggcccgcgggggcccccccgaggccttcaccaccagcgtgcgcagctacctgcccaacacggtgaccgacgcactgcgggggagcggggcgtgggggctgctgctgcgccgcgtgggcgacgacgtgctggttcacctgctggcacgctgcgcgctctttgtgctggtggctcccagctgcgcctaccaggtgtgcgggccgccgctgtaccagctcggcgctgccactcaggcccggcccccgccacacgctagtggaccccgaaggcgtctgggatgcgaacgggcctggaaccatagcgtcagggaggccggggtccccctgggcctgccagccccgggtgcgaggaggcgcgggggcagtgccagccgaagtctgccgttgcccaagaggcccaggcgtggcgctgcccctgagccggagcggacgcccgttgggcaggggtcctgggcccacccgggcaggacgcgtggaccgagtgaccgtggtttctgtgtggtgtcacctgccagacccgccgaagaagccacctctttggagggtgcgctctctggcacgcgccactcccacccatccgtgggccgccagcaccacgcgggccccccatccacatcgcggccaccacgtccctgggacacgccttgtcccccggtgtacgccgagaccaagcacttcctctactcctcaggcgacaaggagcagctgcggccctccttcctactcagctctctgaggcccagcctgactggcgctcggaggctcgtggagaccatctttctgggttccaggccctggatgccagggactccccgcaggttgccccgcctgccccagcgctactggcaaatgcggcccctgtttctggagctgcttgggaaccacgcgcagtgcccctacggggtgctcctcaagacgcactgcccgctgcgagctgcggtcaccccagcagccggtgtctgtgcccgggagaagccccagggctctgtggcggcccccgaggaggaggacacagacccccgtcgcctggtgcagctgctccgccagcacagcagcccctggcaggtgtacggcttcgtgcgggcctgcctgcgccggctggtgcccccaggcctctggggctccaggcacaacgaacgccgcttcctcaggaacaccaagaagttcatctccctggggaagcatgccaagctctcgctgcaggagctgacgtggaagatgagcgtgcgggactgcgcttggctgcgcaggagcccaggggttggctgtgttccggccgcagagcaccgtctgcgtgaggagatcctggccaagttcctgcactggctgatgagtgtgtacgtcgtcgagctgctcaggtctttcttttatgtcacggagaccacgtttcaaaagaacaggctctttttctaccggaagagtgtctggagcaagttgcaaagcattggaatcagacagcacttgaagagggtgcagctgcgggagctgtcggaagcagaggtcaggcagcatcgggaagccaggcccgccctgctgacgtccagactccgcttcatccccaagcctgacgggctgcggccgattgtgaacatggactacgtcgtgggagccagaacgttccgcagagaaaagagggccgagcgtctcacctcgagggtgaaggcactgttcagcgtgctcaactacgagcgggcgcggcgccccggcctcctgggcgcctctgtgctgggcctggacgatatccacagggcctggcgcaccttcgtgctgcgtgtgcgggcccaggacccgccgcctgagctgtactttgtcaaggtggatgtgacgggcgcgtacgacaccatcccccaggacaggctcacggaggtcatcgccagcatcatcaaaccccagaacacgtactgcgtgcgtcggtatgccgtggtccagaaggccgcccatgggcacgtccgcaaggccttcaagagccacgtctctaccttgacagacctccagccgtacatgcgacagttcgtggctcacctgcaggagaccagcccgctgagggatgccgtcgtcatcgagcagagctcctccctgaatgaggccagcagtggcctcttcgacgtcttcctacgcttcatgtgccaccacgccgtgcgcatcaggggcaagtcctacgtccagtgccaggggatcccgcagggctccatcctctccacgctgctctgcagcctgtgctacggcgacatggagaacaagctgtttgcggggattcggcgggacgggctgctcctgcgtttggtggatgatttcttgttggtgacacctcacctcacccacgcgaaaaccttcctcaggaccctggtccgaggtgtccctgagtatggctgcgtggtgaacttgcggaagacagtggtgaacttccctgtagaagacgaggccctgggtggcacggcttttgttcagatgccggcccacggcctattcccctggtgcggcctgctgctggatacccggaccctggaggtgcagagcgactactccagctatgcccggacctccatcagagccagtctcaccttcaaccgcggcttcaaggctgggaggaacatgcgtcgcaaactctttggggtcttgcggctgaagtgtcacagcctgtttctggatttgcaggtgaacagcctccagacggtgtgcaccaacatctacaagatcctcctgctgcaggcgtacaggtttcacgcatgtgtgctgcagctcccatttcatcagcaagtttggaagaaccccacatttttcctgcgcgtcatctctgacacggcctccctctgctactccatcctgaaagccaagaacgcagggatgtcgctgggggccaagggcgccgccggccctctgccctccgaggccgtgcagtggctgtgccaccaagcattcctgctcaagctgactcgacaccgtgtcacctacgtgccactcctggggtcactcaggacagcccagacgcagctgagtcggaagctcccggggacgacgctgactgccctggaggccgcagccaacccggcactgccctcagacttcaagaccatcctggactgatctagaggcgcgcc

SEQ ID NO: 16 - DNA, 9354 bp, Artificial Sequence; identical to SEQ ID NO: 10
  synthesis

SEQ ID NO: 17 - DNA, 9162 bp, Artificial Sequence; identical to SEQ ID NO: 9
  synthesis

SEQ ID NO: 18 - DNA, 8568 bp, Artificial Sequence
  synthesis
gtcgacactagtaatcaacctctggattacaaaatttgtgaaagattgactggtattcttaactatgttgctccttttacgctatgtggatacgctgctttaatgcctttgtatcatgctattgcttcccgtatggctttcattttctcctccttgtataaatcctggttgctgtctctttatgaggagttgtggcccgttgtcaggcaacgtggcgtggtgtgcactgtgtttgctgacgcaacccccactggttggggcattgccaccacctgtcagctcctttccgggactttcgctttccccctccctattgccacggcggaactcatcgccgcctgccttgcccgctgctggacaggggctcggctgttgggcactgacaattccgtggtgttgtcggggaagctgacgtcctttccatggctgctcgcctgtgttgccacctggattctgcgcgggacgtccttctgctacgtcccttcggccctcaatccagcggaccttccttcccgcggcctgctgccggctctgcggcctcttccgcgtcttcgccttcgccctcagacgagtcggatctccctttgggccgcctccccgcctgccgcggaattcgagctcggtacctttaagaccaatgacttacaaggcagctgtagatcttagccactttttaaaagaaaaggggggactggaagggctaattcactcccaacgaagacaagatctgctttttgcttgtactgagtctctctggttagaccagatctgagcctgggagctctctggctaactagggaacccactgcttaagcctcaataaagcttgccttgagtgcttcaagtagtgtgtgcccgtctgttgtgtgactctggtaactagagatccctcagacccttttagtcagtgtggaaaatctctagcagtagtagttcatgtcatcttattattcagtatttataacttgcaaagaaatgaatatcagagagtgagaggaacttgtttattgcagcttataatggttacaaataaagcaatagcatcacaaatttcacaaataaagcatttttttcactgcattctagttgtggtttgtccaaactcatcaatgtatcttatcatgtctggctctagctatcccgcccctaactccgcccatcccgcccctaactccgcccagttccgcccattctccgccccatggctgactaattttttttatttatgcagaggccgaggccgcctcggcctctgagctattccagaagtagtgaggaggcttttttggaggcctagggacgtacccaattcgccctatagtgagtcgtattacgcgcgctcactggccgtcgttttacaacgtcgtgactgggaaaaccctggcgttacccaacttaatcgccttgcagcacatccccctttcgccagctggcgtaatagcgaagaggcccgcaccgatcgcccttcccaacagttgcgcagcctgaatggcgaatgggacgcgccctgtagcggcgcattaagcgcggcgggtgtggtggttacgcgcagcgtgaccgctacacttgccagcgccctagcgcccgctcctttcgctttcttcccttcctttctcgccacgttcgccggctttccccgtcaagctctaaatcgggggctccctttagggttccgatttagtgctttacggcacctcgaccccaaaaaacttgattagggtgatggttcacgtagtgggccatcgccctgatagacggtttttcgccctttgacgttggagtccacgttctttaatagtggactcttgttccaaactggaacaacactcaaccctatctcggtctattcttttgatttataagggattttgccgatttcggcctattggttaaaaaatgagctgatttaacaaaaatttaacgcgaattttaacaaaatattaacgcttacaatttaggtggcacttttcggggaaatgtgcgcggaacccctatttgtttatttttctaaatacattcaaatatgtatccgctcatgagacaataaccctgataaatgcttcaataatattgaaaaaggaagagtatgagtattcaacatttccgtgtcgcccttattcccttttttgcggcattttgccttcctgtttttgctcacccagaaacgctggtgaaagtaaaagatgctgaagatcagttgggtgcacgagtgggttacatcgaactggatctcaacagcggtaagatccttgagagttttcgccccgaagaacgttttccaatgatgagcacttttaaagttctgctatgtggcgcggtattatcccgtattgacgccgggcaagagcaactcggtcgccgcatacactattctcagaatgacttggttgagtactcaccagtcacagaaaagcatcttacggatggcatgacagtaagagaattatgcagtgctgccataaccatgagtgataacactgcggccaacttacttctgacaacgatcggaggaccgaaggagctaaccgcttttttgcacaacatgggggatcatgtaactcgccttgatcgttgggaaccggagctgaatgaagccataccaaacgacgagcgtgacaccacgatgcctgtagcaatggcaacaacgttgcgcaaactattaactggcgaactacttactctagcttcccggcaacaattaatagactggatggaggcggataaagttgcaggaccacttctgcgctcggcccttccggctggctggtttattgctgataaatctggagccggtgagcgtggctctcgcggtatcattgcagcactggggccagatggtaagccctcccgtatcgtagttatctacacgacggggagtcaggcaactatggatgaacgaaatagacagatcgctgagataggtgcctcactgattaagcattggtaactgtcagaccaagtttactcatatatactttagattgatttaaaacttcatttttaatttaaaaggatctaggtgaagatcctttttgataatctcatgaccaaaatcccttaacgtgagttttcgttccactgagcgtcagaccccgtagaaaagatcaaaggatcttcttgagatcctttttttctgcgcgtaatctgctgcttgcaaacaaaaaaaccaccgctaccagcggtggtttgtttgccggatcaagagctaccaactctttttccgaaggtaactggcttcagcagagcgcagataccaaatactgttcttctagtgtagccgtagttaggccaccacttcaagaactctgtagcaccgcctacatacctcgctctgctaatcctgttaccagtggctgctgccagtggcgataagtcgtgtcttaccgggttggactcaagacgatagttaccggataaggcgcagcggtcgggctgaacggggggttcgtgcacacagcccagcttggagcgaacgacctacaccgaactgagatacctacagcgtgagctatgagaaagcgccacgcttcccgaagggagaaaggcggacaggtatccggtaagcggcagggtcggaacaggagagcgcacgagggagcttccagggggaaacgcctggtatctttatagtcctgtcgggtttcgccacctctgacttgagcgtcgatttttgtgatgctcgtcaggggggcggagcctatggaaaaacgccagcaacgcggcctttttacggttcctggccttttgctggccttttgctcacatgttctttcctgcgttatcccctgattctgtggataaccgtattaccgcctttgagtgagctgataccgctcgccgcagccgaacgaccgagcgcagcgagtcagtgagcgaggaagcggaagagcgcccaatacgcaaaccgcctctccccgcgcgttggccgattcattaatgcagctggcacgacaggtttcccgactggaaagcgggcagtgagcgcaacgcaattaatgtgagttagctcactcattaggcaccccaggctttacactttatgcttccggctcgtatgttgtgtggaattgtgagcggataacaatttcacacaggaaacagctatgaccatgattacgccaagcgcgcaattaaccctcactaaagggaacaaaagctggagctgcaagcttaatgtagtcttatgcaatactcttgtagtcttgcaacatggtaacgatgagttagcaacatgccttacaaggagagaaaaagcaccgtgcatgccgattggtggaagtaaggtggtacgatcgtgccttattaggaaggcaacagacgggtctgacatggattggacgaaccactgaattgccgcattgcagagatattgtatttaagtgcctagctcgatacataaacggctctctctggttagaccagatctgagcctgggagctctctggctaactagggaacccactgcttaagcctcaataaagcttgccttgagtgcttcaagtagtgtgtgcccgtctgttgtgtgactctggtaactagagatccctcagacccttttagtcagtgtggaaaatctctagcagtggcgcccgaacagggacttgaaagcgaaagggaaaccagaggagctctctcgacgcaggactcggcttgctgaagcgcgcacggcaagaggcgaggggcggcgactggtgagtacgccaaaaattttgactagcggaggctagaaggagagagatgggtgcgagagcgtcagtattaagcgggggagaattagatcgcgatgggaaaaaattcggttaaggccagggggaaagaaaaaatataaattaaaacatatagtatgggcaagcagggagctagaacgattcgcagttaatcctggcctgttagaaacatcagaaggctgtagacaaatactgggacagctacaaccatcccttcagacaggatcagaagaacttagatcattatataatacagtagcaaccctctattgtgtgcatcaaaggatagagataaaagacaccaaggaagctttagacaagatagaggaagagcaaaacaaaagtaagaccaccgcacagcaagcggccgctgatcttcagacctggaggaggagatatgagggacaattggagaagtgaattatataaatataaagtagtaaaaattgaaccattaggagtagcacccaccaaggcaaagagaagagtggtgcagagagaaaaaagagcagtgggaataggagctttgttccttgggttcttgggagcagcaggaagcactatgggcgcagcgtcaatgacgctgacggtacaggccagacaattattgtctggtatagtgcagcagcagaacaatttgctgagggctattgaggcgcaacagcatctgttgcaactcacagtctggggcatcaagcagctccaggcaagaatcctggctgtggaaagatacctaaaggatcaacagctcctggggatttggggttgctctggaaaactcatttgcaccactgctgtgccttggaatgctagttggagtaataaatctctggaacagatttggaatcacacgacctggatggagtgggacagagaaattaacaattacacaagcttaatacactccttaattgaagaatcgcaaaaccagcaagaaaagaatgaacaagaattattggaattagataaatgggcaagtttgtggaattggtttaacataacaaattggctgtggtatataaaattattcataatgatagtaggaggcttggtaggtttaagaatagtttttgctgtactttctatagtgaatagagttaggcagggatattcaccattatcgtttcagacccacctcccaaccccgaggggacccgacaggcccgaaggaatagaagaagaaggtggagagagagacagagacagatccattcgattagtgaacggatctcgacggtatcgatcacgagactagcctcgacacaaatggcagtattcatccacaattttaaaagaaaaggggggattggggggtacagtgcaggggaaagaatagtagacataatagcaacagacatacaaactaaagaattacaaaaacaaattacaaaaattcaaaattttcgggtttattacagggacagcagaaatccactttggctcgagaagcttgatatcggctccggtgcccgtcagtgggcagagcgcacatcgcccacagtccccgagaagttggggggaggggtcggcaattgaaccggtgcctagagaaggtggcgcggggtaaactgggaaagtgatgtcgtgtactggctccgcctttttcccgagggtgggggagaaccgtatataagtgcagtagtcgccgtgaacgttctttttcgcaacgggtttgccgccagaacacaggatccgccaccatggataaagttttaaacagagaggaatctttgcagctaatggaccttctaggtcttgaaaggagtgcctgggggaatattcctctgatgagaaaggcatatttaaaaaaatgcaaggagtttcatcctgataaaggaggagatgaagaaaaaatgaagaaaatgaatactctgtacaagaaaatggaagatggagtaaaatatgctcatcaacctgactttggaggcttctgggatgcaactgagattccaacctatggaactgatgaatgggagcagtggtggaatgcctttaatgaggaaaacctgttttgctcagaagaaatgccatctagtgatgatgaggctactgctgactctcaacattctactcctccaaaaaagaagagaaaggtagaagaccccaaggactttccttcagaattgctaagttttttgagtcatgctgtgtttagtaatagaactcttgcttgctttgctatttacaccacaaaggaaaaagctgcactgctatacaagaaaattatggaaaaatattctgtaacctttataagtaggcataacagttataatcataacatactgttttttcttactccacacaggcatagagtgtctgctattaataactatgctcaaaaattgtgtacctttagctttttaatttgtaaaggggttaataaggaatatttgatgtatagtgccttgactagagatccattttctgttattgaggaaagtttgccaggtgggttaaaggagcatgattttaatccagaagaagcagaggaaactaaacaagtgtcctggaagcttgtaacagagtatgcaatggaaacaaaatgtgatgatgtgttgttattgcttgggatgtacttggaatttcagtacagttttgaaatgtgtttaaaatgtattaaaaaagaacagcccagccactataagtaccatgaaaagcattatgcaaatgctgctatatttgctgacagcaaaaaccaaaaaaccatatgccaacaggctgttgatactgttttagctaaaaagcgggttgatagcctacaattaactagagaacaaatgttaacaaacagatttaatgatcttttggataggatggatataatgtttggttctacaggctctgctgacatagaagaatggatggctggagttgcttggctacactgtttgttgcccaaaatggattcagtggtgtatgactttttaaaatgcatggtgtacaacattcctaaaaaaagatactggctgtttaaaggaccaattgatagtggtaaaactacattagcagctgctttgcttgaattatgtggggggaaagctttaaatgttaatttgcccttggacaggctgaactttgagctaggagtagctattgaccagtttttagtagtttttgaggatgtaaagggcactggaggggagtccagagatttgccttcaggtcagggaattaataacctggacaatttaagggattatttggatggcagtgttaaggtaaacttagaaaagaaacacctaaataaaagaactcaaatatttccccctggaatagtcaccatgaatgagtacagtgtgcctaaaacactgcaggccagatttgtaaaacaaatagattttaggcccaaagattatttaaagcattgcctggaacgcagtgagtttttgttagaaaagagaataattcaaagtggcattgctttgcttcttatgttaatttggtacagacctgtggctgagtttgctcaaagtattcagagcagaattgtggagtggaaagagagattggacaaagagtttagtttgtcagtgtatcaaaaaatgaagtttaatgtggctatgggaattggagttttagattggctaagaaacagtgatgatgatgatgaagacagccaggaaaatgctgataaaaatgaagatggtggggagaagaacatggaagactcagggcatgaaacaggcattgattcacagtcccaaggctcatttcaggcccctcagtcctcacagtctgttcatgatcataatcagccataccacatttgtagaggttttacttgctttaaaaaacctcccacacctccccctgaacctgaaacataatctagaggcgcgcc

SEQ ID NO: 19 - DNA, 7914 bp, Artificial Sequence
  synthesis
gtcgacactagtaatcaacctctggattacaaaatttgtgaaagattgactggtattcttaactatgttgctccttttacgctatgtggatacgctgctttaatgcctttgtatcatgctattgcttcccgtatggctttcattttctcctccttgtataaatcctggttgctgtctctttatgaggagttgtggcccgttgtcaggcaacgtggcgtggtgtgcactgtgtttgctgacgcaacccccactggttggggcattgccaccacctgtcagctcctttccgggactttcgctttccccctccctattgccacggcggaactcatcgccgcctgccttgcccgctgctggacaggggctcggctgttgggcactgacaattccgtggtgttgtcggggaagctgacgtcctttccatggctgctcgcctgtgttgccacctggattctgcgcgggacgtccttctgctacgtcccttcggccctcaatccagcggaccttccttcccgcggcctgctgccggctctgcggcctcttccgcgtcttcgccttcgccctcagacgagtcggatctccctttgggccgcctccccgcctgccgcggaattcgagctcggtacctttaagaccaatgacttacaaggcagctgtagatcttagccactttttaaaagaaaaggggggactggaagggctaattcactcccaacgaagacaagatctgctttttgcttgtactgagtctctctggttagaccagatctgagcctgggagctctctggctaactagggaacccactgcttaagcctcaataaagcttgccttgagtgcttcaagtagtgtgtgcccgtctgttgtgtgactctggtaactagagatccctcagacccttttagtcagtgtggaaaatctctagcagtagtagttcatgtcatcttattattcagtatttataacttgcaaagaaatgaatatcagagagtgagaggaacttgtttattgcagcttataatggttacaaataaagcaatagcatcacaaatttcacaaataaagcatttttttcactgcattctagttgtggtttgtccaaactcatcaatgtatcttatcatgtctggctctagctatcccgcccctaactccgcccatcccgcccctaactccgcccagttccgcccattctccgccccatggctgactaattttttttatttatgcagaggccgaggccgcctcggcctctgagctattccagaagtagtgaggaggcttttttggaggcctagggacgtacccaattcgccctatagtgagtcgtattacgcgcgctcactggccgtcgttttacaacgtcgtgactgggaaaaccctggcgttacccaacttaatcgccttgcagcacatccccctttcgccagctggcgtaatagcgaagaggcccgcaccgatcgcccttcccaacagttgcgcagcctgaatggcgaatgggacgcgccctgtagcggcgcattaagcgcggcgggtgtggtggttacgcgcagcgtgaccgctacacttgccagcgccctagcgcccgctcctttcgctttcttcccttcctttctcgccacgttcgccggctttccccgtcaagctctaaatcgggggctccctttagggttccgatttagtgctttacggcacctcgaccccaaaaaacttgattagggtgatggttcacgtagtgggccatcgccctgatagacggtttttcgccctttgacgttggagtccacgttctttaatagtggactcttgttccaaactggaacaacactcaaccctatctcggtctattcttttgatttataagggattttgccgatttcggcctattggttaaaaaatgagctgatttaacaaaaatttaacgcgaattttaacaaaatattaacgcttacaatttaggtggcacttttcggggaaatgtgcgcggaacccctatttgtttatttttctaaatacattcaaatatgtatccgctcatgagacaataaccctgataaatgcttcaataatattgaaaaaggaagagtatgagtattcaacatttccgtgtcgcccttattcccttttttgcggcattttgccttcctgtttttgctcacccagaaacgctggtgaaagtaaaagatgctgaagatcagttgggtgcacgagtgggttacatcgaactggatctcaacagcggtaagatccttgagagttttcgccccgaagaacgttttccaatgatgagcacttttaaagttctgctatgtggcgcggtattatcccgtattgacgccgggcaagagcaactcggtcgccgcatacactattctcagaatgacttggttgagtactcaccagtcacagaaaagcatcttacggatggcatgacagtaagagaattatgcagtgctgccataaccatgagtgataacactgcggccaacttacttctgacaacgatcggaggaccgaaggagctaaccgcttttttgcacaacatgggggatcatgtaactcgccttgatcgttgggaaccggagctgaatgaagccataccaaacgacgagcgtgacaccacgatgcctgtagcaatggcaacaacgttgcgcaaactattaactggcgaactacttactctagcttcccggcaacaattaatagactggatggaggcggataaagttgcaggaccacttctgcgctcggcccttccggctggctggtttattgctgataaatctggagccggtgagcgtggctctcgcggtatcattgcagcactggggccagatggtaagccctcccgtatcgtagttatctacacgacggggagtcaggcaactatggatgaacgaaatagacagatcgctgagataggtgcctcactgattaagcattggtaactgtcagaccaagtttactcatatatactttagattgatttaaaacttcatttttaatttaaaaggatctaggtgaagatcctttttgataatctcatgaccaaaatcccttaacgtgagttttcgttccactgagcgtcagaccccgtagaaaagatcaaaggatcttcttgagatcctttttttctgcgcgtaatctgctgcttgcaaacaaaaaaaccaccgctaccagcggtggtttgtttgccggatcaagagctaccaactctttttccgaaggtaactggcttcagcagagcgcagataccaaatactgttcttctagtgtagccgtagttaggccaccacttcaagaactctgtagcaccgcctacatacctcgctctgctaatcctgttaccagtggctgctgccagtggcgataagtcgtgtcttaccgggttggactcaagacgatagttaccggataaggcgcagcggtcgggctgaacggggggttcgtgcacacagcccagcttggagcgaacgacctacaccgaactgagatacctacagcgtgagctatgagaaagcgccacgcttcccgaagggagaaaggcggacaggtatccggtaagcggcagggtcggaacaggagagcgcacgagggagcttccagggggaaacgcctggtatctttatagtcctgtcgggtttcgccacctctgacttgagcgtcgatttttgtgatgctcgtcaggggggcggagcctatggaaaaacgccagcaacgcggcctttttacggttcctggccttttgctggccttttgctcacatgttctttcctgcgttatcccctgattctgtggataaccgtattaccgcctttgagtgagctgataccgctcgccgcagccgaacgaccgagcgcagcgagtcagtgagcgaggaagcggaagagcgcccaatacgcaaaccgcctctccccgcgcgttggccgattcattaatgcagctggcacgacaggtttcccgactggaaagcgggcagtgagcgcaacgcaattaatgtgagttagctcactcattaggcaccccaggctttacactttatgcttccggctcgtatgttgtgtggaattgtgagcggataacaatttcacacaggaaacagctatgaccatgattacgccaagcgcgcaattaaccctcactaaagggaacaaaagctggagctgcaagcttaatgtagtcttatgcaatactcttgtagtcttgcaacatggtaacgatgagttagcaacatgccttacaaggagagaaaaagcaccgtgcatgccgattggtggaagtaaggtggtacgatcgtgccttattaggaaggcaacagacgggtctgacatggattggacgaaccactgaattgccgcattgcagagatattgtatttaagtgcctagctcgatacataaacggctctctctggttagaccagatctgagcctgggagctctctggctaactagggaacccactgcttaagcctcaataaagcttgccttgagtgcttcaagtagtgtgtgcccgtctgttgtgtgactctggtaactagagatccctcagacccttttagtcagtgtggaaaatctctagcagtggcgcccgaacagggacttgaaagcgaaagggaaaccagaggagctctctcgacgcaggactcggcttgctgaagcgcgcacggcaagaggcgaggggcggcgactggtgagtacgccaaaaattttgactagcggaggctagaaggagagagatgggtgcgagagcgtcagtattaagcgggggagaattagatcgcgatgggaaaaaattcggttaaggccagggggaaagaaaaaatataaattaaaacatatagtatgggcaagcagggagctagaacgattcgcagttaatcctggcctgttagaaacatcagaaggctgtagacaaatactgggacagctacaaccatcccttcagacaggatcagaagaacttagatcattatataatacagtagcaaccctctattgtgtgcatcaaaggatagagataaaagacaccaaggaagctttagacaagatagaggaagagcaaaacaaaagtaagaccaccgcacagcaagcggccgctgatcttcagacctggaggaggagatatgagggacaattggagaagtgaattatataaatataaagtagtaaaaattgaaccattaggagtagcacccaccaaggcaaagagaagagtggtgcagagagaaaaaagagcagtgggaataggagctttgttccttgggttcttgggagcagcaggaagcactatgggcgcagcgtcaatgacgctgacggtacaggccagacaattattgtctggtatagtgcagcagcagaacaatttgctgagggctattgaggcgcaacagcatctgttgcaactcacagtctggggcatcaagcagctccaggcaagaatcctggctgtggaaagatacctaaaggatcaacagctcctggggatttggggttgctctggaaaactcatttgcaccactgctgtgccttggaatgctagttggagtaataaatctctggaacagatttggaatcacacgacctggatggagtgggacagagaaattaacaattacacaagcttaatacactccttaattgaagaatcgcaaaaccagcaagaaaagaatgaacaagaattattggaattagataaatgggcaagtttgtggaattggtttaacataacaaattggctgtggtatataaaattattcataatgatagtaggaggcttggtaggtttaagaatagtttttgctgtactttctatagtgaatagagttaggcagggatattcaccattatcgtttcagacccacctcccaaccccgaggggacccgacaggcccgaaggaatagaagaagaaggtggagagagagacagagacagatccattcgattagtgaacggatctcgacggtatcgatcacgagactagcctcgacacaaatggcagtattcatccacaattttaaaagaaaaggggggattggggggtacagtgcaggggaaagaatagtagacataatagcaacagacatacaaactaaagaattacaaaaacaaattacaaaaattcaaaattttcgggtttattacagggacagcagaaatccactttggctcgagaagcttgatatcggctccggtgcccgtcagtgggcagagcgcacatcgcccacagtccccgagaagttggggggaggggtcggcaattgaaccggtgcctagagaaggtggcgcggggtaaactgggaaagtgatgtcgtgtactggctccgcctttttcccgagggtgggggagaaccgtatataagtgcagtagtcgccgtgaacgttctttttcgcaacgggtttgccgccagaacacaggatccgccaccatggccttaccagtgaccgccttgctcctgccgctggccttgctgctccacgccgccaggccggatatccagatgacccagagcccaagctccctgtccgcctctgtgggcgacagggtgaccatcacatgccgcgccagccagacaatctggtcctacctgaactggtatcagcagagacccggcaaggcccctaatctgctgatctacgcagcatctagcctgcagtctggagtgccctcccggttctctggaagaggatccggaaccgacttcaccctgacaatctcctctctgcaggccgaggacttcgccacatactattgccagcagagctattccatccctcagacctttggccagggcacaaagctggagatcaagggcggcggcggctctggaggaggaggaagcggaggaggaggatcccaggtgcagctgcagcagagcggaccaggactggtgaagccctcccagaccctgtctctgacatgtgccatcagcggcgattccgtgagctccaacagcgccgcctggaattggatccggcagtctcccagcagaggactggagtggctgggaaggacctactatcgctccaagtggtacaacgattatgccgtgtctgtgaagagccggatcaccatcaaccctgacacatctaagaatcagttcagcctgcagctgaattccgtgaccccagaggacacagccgtgtactattgtgcaagggaggtgaccggcgacctggaggatgcctttgacatctggggccagggcaccatggtgacagtgtctagcaccacgacgccagcgccgcgaccaccaacaccggcgcccaccatcgcgtcgcagcccctgtccctgcgcccagaggcgtgccggccagcggcggggggcgcagtgcacacgagggggctggacttcgcctgtgatatctacatctgggcgcccttggccgggacttgtggggtccttctcctgtcactggttatcaccctttactgcaaacggggcagaaagaaactcctgtatatattcaaacaaccatttatgagaccagtacaaactactcaagaggaagatggctgtagctgccgatttccagaagaagaagaaggaggatgtgaactgagagtgaagttcagcaggagcgcagacgcccccgcgtacaagcagggccagaaccagctctataacgagctcaatctaggacgaagagaggagtacgatgttttggacaagaggcgtggccgggaccctgagatggggggaaagccgagaaggaagaaccctcaggaaggcctgtacaatgaactgcagaaagataagatggcggaggcctacagtgagattgggatgaaaggcgagcgccggaggggcaaggggcacgatggcctttaccagggtctcagtacagccaccaaggacacctacgacgcccttcacatgcaggccctgccccctcgctaatctagaggcgcgcc

SEQ ID NO: 20 - DNA, 7899 bp, Artificial Sequence
  synthesis
gtcgacactagtaatcaacctctggattacaaaatttgtgaaagattgactggtattcttaactatgttgctccttttacgctatgtggatacgctgctttaatgcctttgtatcatgctattgcttcccgtatggctttcattttctcctccttgtataaatcctggttgctgtctctttatgaggagttgtggcccgttgtcaggcaacgtggcgtggtgtgcactgtgtttgctgacgcaacccccactggttggggcattgccaccacctgtcagctcctttccgggactttcgctttccccctccctattgccacggcggaactcatcgccgcctgccttgcccgctgctggacaggggctcggctgttgggcactgacaattccgtggtgttgtcggggaagctgacgtcctttccatggctgctcgcctgtgttgccacctggattctgcgcgggacgtccttctgctacgtcccttcggccctcaatccagcggaccttccttcccgcggcctgctgccggctctgcggcctcttccgcgtcttcgccttcgccctcagacgagtcggatctccctttgggccgcctccccgcctgccgcggaattcgagctcggtacctttaagaccaatgacttacaaggcagctgtagatcttagccactttttaaaagaaaaggggggactggaagggctaattcactcccaacgaagacaagatctgctttttgcttgtactgagtctctctggttagaccagatctgagcctgggagctctctggctaactagggaacccactgcttaagcctcaataaagcttgccttgagtgcttcaagtagtgtgtgcccgtctgttgtgtgactctggtaactagagatccctcagacccttttagtcagtgtggaaaatctctagcagtagtagttcatgtcatcttattattcagtatttataacttgcaaagaaatgaatatcagagagtgagaggaacttgtttattgcagcttataatggttacaaataaagcaatagcatcacaaatttcacaaataaagcatttttttcactgcattctagttgtggtttgtccaaactcatcaatgtatcttatcatgtctggctctagctatcccgcccctaactccgcccatcccgcccctaactccgcccagttccgcccattctccgccccatggctgactaattttttttatttatgcagaggccgaggccgcctcggcctctgagctattccagaagtagtgaggaggcttttttggaggcctagggacgtacccaattcgccctatagtgagtcgtattacgcgcgctcactggccgtcgttttacaacgtcgtgactgggaaaaccctggcgttacccaacttaatcgccttgcagcacatccccctttcgccagctggcgtaatagcgaagaggcccgcaccgatcgcccttcccaacagttgcgcagcctgaatggcgaatgggacgcgccctgtagcggcgcattaagcgcggcgggtgtggtggttacgcgcagcgtgaccgctacacttgccagcgccctagcgcccgctcctttcgctttcttcccttcctttctcgccacgttcgccggctttccccgtcaagctctaaatcgggggctccctttagggttccgatttagtgctttacggcacctcgaccccaaaaaacttgattagggtgatggttcacgtagtgggccatcgccctgatagacggtttttcgccctttgacgttggagtccacgttctttaatagtggactcttgttccaaactggaacaacactcaaccctatctcggtctattcttttgatttataagggattttgccgatttcggcctattggttaaaaaatgagctgatttaacaaaaatttaacgcgaattttaacaaaatattaacgcttacaatttaggtggcacttttcggggaaatgtgcgcggaacccctatttgtttatttttctaaatacattcaaatatgtatccgctcatgagacaataaccctgataaatgcttcaataatattgaaaaaggaagagtatgagtattcaacatttccgtgtcgcccttattcccttttttgcggcattttgccttcctgtttttgctcacccagaaacgctggtgaaagtaaaagatgctgaagatcagttgggtgcacgagtgggttacatcgaactggatctcaacagcggtaagatccttgagagttttcgccccgaagaacgttttccaatgatgagcacttttaaagttctgctatgtggcgcggtattatcccgtattgacgccgggcaagagcaactcggtcgccgcatacactattctcagaatgacttggttgagtactcaccagtcacagaaaagcatcttacggatggcatgacagtaagagaattatgcagtgctgccataaccatgagtgataacactgcggccaacttacttctgacaacgatcggaggaccgaaggagctaaccgcttttttgcacaacatgggggatcatgtaactcgccttgatcgttgggaaccggagctgaatgaagccataccaaacgacgagcgtgacaccacgatgcctgtagcaatggcaacaacgttgcgcaaactattaactggcgaactacttactctagcttcccggcaacaattaatagactggatggaggcggataaagttgcaggaccacttctgcgctcggcccttccggctggctggtttattgctgataaatctggagccggtgagcgtggctctcgcggtatcattgcagcactggggccagatggtaagccctcccgtatcgtagttatctacacgacggggagtcaggcaactatggatgaacgaaatagacagatcgctgagataggtgcctcactgattaagcattggtaactgtcagaccaagtttactcatatatactttagattgatttaaaacttcatttttaatttaaaaggatctaggtgaagatcctttttgataatctcatgaccaaaatcccttaacgtgagttttcgttccactgagcgtcagaccccgtagaaaagatcaaaggatcttcttgagatcctttttttctgcgcgtaatctgctgcttgcaaacaaaaaaaccaccgctaccagcggtggtttgtttgccggatcaagagctaccaactctttttccgaaggtaactggcttcagcagagcgcagataccaaatactgttcttctagtgtagccgtagttaggccaccacttcaagaactctgtagcaccgcctacatacctcgctctgctaatcctgttaccagtggctgctgccagtggcgataagtcgtgtcttaccgggttggactcaagacgatagttaccggataaggcgcagcggtcgggctgaacggggggttcgtgcacacagcccagcttggagcgaacgacctacaccgaactgagatacctacagcgtgagctatgagaaagcgccacgcttcccgaagggagaaaggcggacaggtatccggtaagcggcagggtcggaacaggagagcgcacgagggagcttccagggggaaacgcctggtatctttatagtcctgtcgggtttcgccacctctgacttgagcgtcgatttttgtgatgctcgtcaggggggcggagcctatggaaaaacgccagcaacgcggcctttttacggttcctggccttttgctggccttttgctcacatgttctttcctgcgttatcccctgattctgtggataaccgtattaccgcctttgagtgagctgataccgctcgccgcagccgaacgaccgagcgcagcgagtcagtgagcgaggaagcggaagagcgcccaatacgcaaaccgcctctccccgcgcgttggccgattcattaatgcagctggcacgacaggtttcccgactggaaagcgggcagtgagcgcaacgcaattaatgtgagttagctcactcattaggcaccccaggctttacactttatgcttccggctcgtatgttgtgtggaattgtgagcggataacaatttcacacaggaaacagctatgaccatgattacgccaagcgcgcaattaaccctcactaaagggaacaaaagctggagctgcaagcttaatgtagtcttatgcaatactcttgtagtcttgcaacatggtaacgatgagttagcaacatgccttacaaggagagaaaaagcaccgtgcatgccgattggtggaagtaaggtggtacgatcgtgccttattaggaaggcaacagacgggtctgacatggattggacgaaccactgaattgccgcattgcagagatattgtatttaagtgcctagctcgatacataaacggctctctctggttagaccagatctgagcctgggagctctctggctaactagggaacccactgcttaagcctcaataaagcttgccttgagtgcttcaagtagtgtgtgcccgtctgttgtgtgactctggtaactagagatccctcagacccttttagtcagtgtggaaaatctctagcagtggcgcccgaacagggacttgaaagcgaaagggaaaccagaggagctctctcgacgcaggactcggcttgctgaagcgcgcacggcaagaggcgaggggcggcgactggtgagtacgccaaaaattttgactagcggaggctagaaggagagagatgggtgcgagagcgtcagtattaagcgggggagaattagatcgcgatgggaaaaaattcggttaaggccagggggaaagaaaaaatataaattaaaacatatagtatgggcaagcagggagctagaacgattcgcagttaatcctggcctgttagaaacatcagaaggctgtagacaaatactgggacagctacaaccatcccttcagacaggatcagaagaacttagatcattatataatacagtagcaaccctctattgtgtgcatcaaaggatagagataaaagacaccaaggaagctttagacaagatagaggaagagcaaaacaaaagtaagaccaccgcacagcaagcggccgctgatcttcagacctggaggaggagatatgagggacaattggagaagtgaattatataaatataaagtagtaaaaattgaaccattaggagtagcacccaccaaggcaaagagaagagtggtgcagagagaaaaaagagcagtgggaataggagctttgttccttgggttcttgggagcagcaggaagcactatgggcgcagcgtcaatgacgctgacggtacaggccagacaattattgtctggtatagtgcagcagcagaacaatttgctgagggctattgaggcgcaacagcatctgttgcaactcacagtctggggcatcaagcagctccaggcaagaatcctggctgtggaaagatacctaaaggatcaacagctcctggggatttggggttgctctggaaaactcatttgcaccactgctgtgccttggaatgctagttggagtaataaatctctggaacagatttggaatcacacgacctggatggagtgggacagagaaattaacaattacacaagcttaatacactccttaattgaagaatcgcaaaaccagcaagaaaagaatgaacaagaattattggaattagataaatgggcaagtttgtggaattggtttaacataacaaattggctgtggtatataaaattattcataatgatagtaggaggcttggtaggtttaagaatagtttttgctgtactttctatagtgaatagagttaggcagggatattcaccattatcgtttcagacccacctcccaaccccgaggggacccgacaggcccgaaggaatagaagaagaaggtggagagagagacagagacagatccattcgattagtgaacggatctcgacggtatcgatcacgagactagcctcgacacaaatggcagtattcatccacaattttaaaagaaaaggggggattggggggtacagtgcaggggaaagaatagtagacataatagcaacagacatacaaactaaagaattacaaaaacaaattacaaaaattcaaaattttcgggtttattacagggacagcagaaatccactttggctcgagaagcttgatatcggctccggtgcccgtcagtgggcagagcgcacatcgcccacagtccccgagaagttggggggaggggtcggcaattgaaccggtgcctagagaaggtggcgcggggtaaactgggaaagtgatgtcgtgtactggctccgcctttttcccgagggtgggggagaaccgtatataagtgcagtagtcgccgtgaacgttctttttcgcaacgggtttgccgccagaacacaggatccgccaccatggccttaccagtgaccgccttgctcctgccgctggccttgctgctccacgccgccaggccgcggatcgtgatgacccagtctccaggcacactgtctgtgagcccaggagagaccgccacactgtcctgccgggcctcccagtctttcagcaacatgctggcctggtaccagcagaagtccggccagccccctagactgctgatctatggcgtgtctaccagggcagcaggagtgccagcaagattctccggatctggaagcggcacagagtttaccctgacaatctccaatctgcagtctgaggacttcgccgtgtactattgccagcagtacggcgattggcctaggtatacctttggccagggcacaaaggtggagcgcaagggaggaggaggaagcggaggaggaggatccggcggcggcggctctgaggtgcagctggtgcagagcggaggaggagtggtgaggcctggaggatctctgcgcctgccatgtgcagcaagcggcttcacctttgacgattacggaatgagctgggtgaggcaggcaccaggcaagggactggagtgggtgtccggcatcaactggaatggaggaagcaccggatacgcagactccgtgaagggccggttcacaatctctagagataacgccaagaatagcctgtatctgcagatgaactccctgatcgccgaggacaccgccctgtaccactgtgcaaggggaggcgactatgatgcctttgatatctggggccagggcaccatggtgacagtgagctccaccacgacgccagcgccgcgaccaccaacaccggcgcccaccatcgcgtcgcagcccctgtccctgcgcccagaggcgtgccggccagcggcggggggcgcagtgcacacgagggggctggacttcgcctgtgatatctacatctgggcgcccttggccgggacttgtggggtccttctcctgtcactggttatcaccctttactgcaaacggggcagaaagaaactcctgtatatattcaaacaaccatttatgagaccagtacaaactactcaagaggaagatggctgtagctgccgatttccagaagaagaagaaggaggatgtgaactgagagtgaagttcagcaggagcgcagacgcccccgcgtacaagcagggccagaaccagctctataacgagctcaatctaggacgaagagaggagtacgatgttttggacaagaggcgtggccgggaccctgagatggggggaaagccgagaaggaagaaccctcaggaaggcctgtacaatgaactgcagaaagataagatggcggaggcctacagtgagattgggatgaaaggcgagcgccggaggggcaaggggcacgatggcctttaccagggtctcagtacagccaccaaggacacctacgacgcccttcacatgcaggccctgccccctcgctaatctagaggcgcgcc

SEQ ID NO: 21 - protein, 242 aa, Artificial Sequence
  Synthesized
DIQMTQTTSSLSASLGDRVTISCRASQDISKYLNWYQQKPDGTVKLLIYHTSRLHSGVPSRFSGSGSGTDYSLTISNLEQEDIATYFCQQGNTLPYTFGGGTKLEITGGGGSGGGGSGGGGSEVKLQESGPGLVAPSQSLSVTCTVSGVSLPDYGVSWIRQPPRKGLEWLGVIWGSETTYYNSALKSRLTIIKDNSKSQVFLKMNSLQTDDTAIYYCAKHYYYGGSYAMDYWGQGTSVTVSS

SEQ ID NO: 22 - protein, 270 aa, Artificial Sequence
  Synthesized
PEEPLVVKVEEGDNAVLQCLKGTSDGPTQQLTWSRESPLKPFLKLSLGLPGLGIHMRPLAIWLFIFNVSQQMGGFYLCQPGPPSEKAWQPGWTVNVEGSGELFRWNVSDLGGLGCGLKNRSSEGPSSPSGKLMSPKLYVWAKDRPEIWEGEPPCLPPRDSLNQSLSQDLTMAPGSTLWLSCGVPPDSVSRGPLSWTHVHPKGPKSLLSLELKDDRPARDMWVMETGLLLPRATAQDAGKYYCHRGNLTMSFHLEITARPVLWHWLLRTGG

SEQ ID NO: 23 - protein, 196 aa, Artificial Sequence
  Synthesized
QLVKSELEEKKSELRHKLKYVPHEYIELIEIARNSTQDRILEMKVMEFFMKVYGYRGKHLGGSRKPDGAIYTVGSPIDYGVIVDTKAYSGGYNLPIGQADEMQRYVEENQTRNKHINPNEWWKVYPSSVTEFKFLFVSGHFKGNYKAQLTRLNHITNCNGAVLSVEELLIGGEMIKAGTLTLEEVRRKFNNGEINF

SEQ ID NO: 24 - protein, 196 aa, Artificial Sequence
  Synthesized
QLVKSELEEKKSELRHKLKYVPHEYIELIEIARNSTQDRILEMKVMEFFMKVYGYRGKHLGGSRKPDGAIYTVGSPIDYGVIVDTKAYSGGYNLPIGQADEMQRYVKENQTRNKHINPNEWWKVYPSSVTEFKFLFVSGHFKGNYKAQLTRLNHKTNCNGAVLSVEELLIGGEMIKAGTLTLEEVRRKFNNGEINF

SEQ ID NO: 25 - protein, 7 aa, Artificial Sequence
  Synthesized
WRSSLAS

SEQ ID NO: 26 - protein, 7 aa, Artificial Sequence
  Synthesized
QSGDLTR

SEQ ID NO: 27 - protein, 7 aa, Artificial Sequence
  Synthesized
HKWVLRQ

SEQ ID NO: 28 - protein, 7 aa, Artificial Sequence
  Synthesized
CPSNLRR

SEQ ID NO: 29 - DNA, 15 bp, Artificial Sequence
  Synthesized
gactttgcatgtgca

SEQ ID NO: 30 - protein, 7 aa, Artificial Sequence
  Synthesized
ERGTLAR

SEQ ID NO: 31 - protein, 7 aa, Artificial Sequence
  Synthesized
RSDNLRE

SEQ ID NO: 32 - protein, 7 aa, Artificial Sequence
  Synthesized
TSGALTR

SEQ ID NO: 33 - DNA, 13 bp, Artificial Sequence
  Synthesized
gttgctccaggcc

SEQ ID NO: 34 - protein, 380 aa, Artificial Sequence
  Synthesized
MRPADLLQLVLLLDLPRDLGGMGCSSPPCECHQEEDFRVTCKDIQRIPSLPPSTQTLKLIETHLRTIPSHAFSNLPNISRIYVSIDVTLQQLESHSFYNLSKVTHIEIRNTRNLTYIDPDALKELPLLKFLGIFNTGLKMFPDLTKVYSTDIFFILEITDNPYMTSIPVNAFQGLCNETLTLKLYNNGFTSVQGYAFNGTKLDAVYLNKNKYLTVIDKDAFGGVYSGPSLLDVSQTSVTALPSKGLEHLKELIARNTWTLKKLPLSLSFLHLTRADLSYPSHCCAFKNQKKIRGILESLMCNESSMQSLRQRKSVNALNSPLHQEYEENLGDSIVGYKEKSKFQDTHNNAHYYVFFEEQEDEIIGFGQELKNPQEETLQA

SEQ ID NO: 35 - protein, 69 aa, Artificial Sequence
  Synthesized
TTTPAPRPPTPAPTIASQPLSLRPEACRPAAGGAVHTRGLDFACDIYIWAPLAGTCGVLLLSLVITLYC

SEQ ID NO: 36 - protein, 47 aa, Artificial Sequence
  Synthesized
TTTPAPRPPTPAPTIASQPLSLRPEACRPAAGGAVHTRGLDFACDIY

SEQ ID NO: 37 - protein, 22 aa, Artificial Sequence
  Synthesized
IWAPLAGTCGVLLLSLVITLYC

SEQ ID NO: 38 - protein, 21 aa, Artificial Sequence
  Synthesized
MALPVTALLLPLALLLHAARP

SEQ ID NO: 39 - protein, 42 aa, Artificial Sequence
  Synthesized
KRGRKKLLYIFKQPFMRPVQTTQEEDGCSCRFPEEEEGGCEL

SEQ ID NO: 40 - protein, 112 aa, Artificial Sequence
  Synthesized
RVKFSRSADAPAYKQGQNQLYNELNLGRREEYDVLDKRRGRDPEMGGKPRRKNPQEGLYNELQKDKMAEAYSEIGMKGERRRGKGHDGLYQGLSTATKDTYDALHMQALPPR

SEQ ID NO: 41 - protein, 272 aa, Homo sapiens
PEEPLVVKVEEGDNAVLQCLKGTSDGPTQQLTWSRESPLKPFLKLSLGLPGLGIHMRPLAIWLFIFNVSQQMGGFYLCQPGPPSEKAWQPGWTVNVEGSGELFRWNVSDLGGLGCGLKNRSSEGPSSPSGKLMSPKLYVWAKDRPEIWEGEPPCLPPRDSLNQSLSQDLTMAPGSTLWLSCGVPPDSVSRGPLSWTHVHPKGPKSLLSLELKDDRPARDMWVMETGLLLPRATAQDAGKYYCHRGNLTMSFHLEITARPVLWHWLLRTGGWK

SEQ ID NO: 42 - protein, 205 aa, Homo sapiens
ISSMDMERPGDGKCQPIEIPMCKDIGYNMTRMPNLMGHENQREAAIQLHEFAPLVEYGCHGHLRFFLCSLYAPMCTEQVSTPIPACRVMCEQARLKCSPIMEQFNFKWPDSLDCRKLPNKNDPNYLCMEAPNNGSDEPTRGSGLFPPLFRPQRPHSAQEHPLKDGGPGRGGCDNPGKFHHVEKSASCAPLCTPGVDVYWSREDKR

SEQ ID NO: 43 - protein, 393 aa, Homo sapiens
GMGCSSPPCECHQEEDFRVTCKDIQRIPSLPPSTQTLKLIETHLRTIPSHAFSNLPNISRIYVSIDVTLQQLESHSFYNLSKVTHIEIRNTRNLTYIDPDALKELPLLKFLGIFNTGLKMFPDLTKVYSTDIFFILEITDNPYMTSIPVNAFQGLCNETLTLKLYNNGFTSVQGYAFNGTKLDAVYLNKNKYLTVIDKDAFGGVYSGPSLLDVSQTSVTALPSKGLEHLKELIARNTWTLKKLPLSLSFLHLTRADLSYPSHCCAFKNQKKIRGILESLMCNESSMQSLRQRKSVNALNSPLHQEYEENLGDSIVGYKEKSKFQDTHNNAHYYVFFEEQEDEIIGFGQELKNPQEETLQAFDSHYDYTICGDSEDMVCTPKSDEFNPCEDIMG

SEQ ID NO: 44 - protein, 210 aa, Homo sapiens
QLPPGKPEIFKCRSPNKETFTCWWRPGTDGGLPTNYSLTYHREGETLMHECPDYITGGPNSCHFGKQYTSMWRTYIMMVNATNQMGSSFSDELYVDVTYIVQPDPPLELAVEVKQPEDRKPYLWIKWSPPTLIDLKTGWFTLLYEIRLKPEKAAEWEIHFAGQQTEFKILSLHPGQKYLVQVRCKPDHGYWSAWSPATFIQIPSDFTMND

SEQ ID NO: 45 - protein, 660 aa, Homo sapiens
EQDLSVNRAVWDGGGCISQGDVLNRQCQQLSQHVRTGSAANTATGTTSTNVVEPRMYLSCSTNPEMTSIESSVTSDTPGVSSTRMTPTESRTTSESTSDSTTLFPSSTEDTSSPTTPEGTDVPMSTPSEESISSTMAFVSTAPLPSFEAYTSLTYKVDMSTPLTTSTQASSSPTTPESTTIPKSTNSEGSTPLTSMPASTMKVASSEAITLLTTPVEISTPVTISAQASSSPTTAEGPSLSNSAPSGGSTPLTRMPLSVMLVVSSEASTLSTTPAATNIPVITSTEASSSPTTAEGTSIPTSTYTEGSTPLTSTPASTMPVATSEMSTLSITPVDTSTLVTTSTEPSSLPTTAEATSMLTSTLSEGSTPLTNMPVSTILVASSEASTTSTIPVDSKTFVTTASEASSSPTTAEDTSIATSTPSEGSTPLTSMPVSTTPVASSEASNLSTTPVDSKTQVTTSTEASSSPPTAEVNSMPTSTPSEGSTPLTSMSVSTMPVASSEASTLSTTPVDTSTPVTTSSEASSSSTTPEGTSIPTSTPSEGSTPLTNMPVSTRLVVSSEASTTSTTPADSNTFVTTSSEASSSSTTAEGTSMPTSTYSERGTTITSMSVSTTLVASSEASTLSTTPVDSNTPVTTSTEATSSSTTAEGTSMPTSTYTE

SEQ ID NO: 46 - protein, 407 aa, Homo sapiens
SQVSQNCHNGSYEISVLMMGNSAFAEPLKNLEDAVNEGLEIVRGRLQNAGLNVTVNATFMYSDGLIHNSGDCRSSTCEGLDLLRKISNAQRMGCVLIGPSCTYSTFQMYLDTELSYPMISAGSFGLSCDYKETLTRLMSPARKLMYFLVNFWKTNDLPFKTYSWSTSYVYKNGTETEDCFWYLNALEASVSYFSHELGFKVVLRQDKEFQDILMDHNRKSNVIIMCGGPEFLYKLKGDRAVAEDIVIILVDLFNDQYFEDNVTAPDYMKNVLVLTLSPGNSLLNSSFSRNLSPTKRDFALAYLNGILLFGHMLKIFLENGENITTPKFAHAFRNLTFEGYDGPVTLDDWGDVDSTMVLLYTSVDTKKYKVLLTYDTHVNKTYPVDMSPTFTWKNSKLPNDITGRGPQ

SEQ ID NO: 47 - protein, 264 aa, Homo sapiens
PRFMGTISDVKTNVQLLKGRVDNISTLDSEIKKNSDGMEAAGVQIQMVNESLGYVRSQFLKLKTSVEKANAQIQILTRSWEEVSTLNAQIPELKSDLEKASALNTKIRALQGSLENMSKLLKRQNDILQVVSQGWKYFKGNFYYFSLIPKTWYSAEQFCVSRNSHLTSVTSESEQEFLYKTAGGLIYWIGLTKAGMEGDWSWVDDTPFNKVQSVRFWIPGEPNNAGNNEHCGNIKAPSLQAWNDAPCDKTFLFICKRPYVPSEP

SEQ ID NO: 48 - protein, 237 aa, Artificial Sequence
  Synthesized
DIQMTQSPASLSVSVGETVTITCRASENIYSNLAWYQQKQGKSPQLLVYVATNLADGVPSRFSGSGSGTQYSLKINSLQSEDFGSYYCQHFWGTPYTFGGGTKLGGGGSGGGGSGGGGSEVQLQQSGAELVKPGASVKLSCTASGFNINDTYMHWVKQRPEQGLEWIGRIDPANGNTKYDPKFQGKATITADTSSNTAYLQLSSLTSEDTAVYYCARGARGSRFAYWGQGTLVTVSA

SEQ ID NO: 49 - protein, 244 aa, Artificial Sequence
  Synthesized
QSVLTQPPSVSAAPGQKVTISCSGSSSDIGSNYVSWYQQFPGTAPKLLIYDNNKRPSAIPDRFSGSKSGTSATLGITGLQTGDEADYYCGTWDSRLGIAVFGGGTQLTVLGGGGSGGGGSGGGGSEVQLVQSGAEVKKPGQSLKISCKASGYSLTDNWIGWVRQKPGKGLEWMGIIYPGDSDTRYSPSFQGQVTISADKSINTAYLQWSSLKASDTAIYYCVGLDWNYNPLRYWGPGTLVTVSS

SEQ ID NO: 50 - protein, 252 aa, Artificial Sequence
  Synthesized
DIVLTQSPASLAVSLGQGATISCRASKSVSTSGYTYMHWYQQKPGQPPKLLIYLASNLESGVPARFSGSGSGTDFTLNIHPVEEEDAATYYCQHSGELPPSFGGGTKLEIKRAGGGGSGGGGSGGGGSEVQLVESGGDLVKPGGSLKLSCAVSGFTFSSYGMSWVRQTPDKRLEWVATVSSGGTYTYYPDSVKGRFTISRDNAKNTLYLQMSSLKSEDSAMYYCARHRGNYYATYYYAMDYWGQGTSVTVSS

SEQ ID NO: 51 - protein, 243 aa, Artificial Sequence
  Synthesized
DVQITQSPSYLAASPGETITINCRASKSISKYLAWYQEKPGKTNKLLIYSGSTLQSGIPSRFSGSGSGTDFTLTISSLEPEDFAMYYCQQHHEYPYTFGGGTKLEIKGGGGSGGGGSGGGGSQVQLQQPGAELVRPGASVKLSCKASGYTFTTYWMNWVKQRPEQGLEWIGRIDPYDSETHYNQKFKDKAILTVDKSSSTAYMQLSSLTSEDSAVYYCARGPYYGTNPWFPYWGQGTLVTVSS

SEQ ID NO: 52 - protein, 241 aa, Artificial Sequence
  Synthesized
EIVMTQSPATLSVSPGERATLSCRASQSVSRNLAWYQQKPGQAPRLLIYGASTRATGIPARFSGSGSGTEFTLTIGSLQSEDFAVYYCQQYKTWPRTFGQGTNVEIKGGGGSGGGGSGGGGSQVQLQQWGAGLLKPSETLSLTCAVFGGSFSGYYWSWIRQPPGKGLEWIGEINHRGNTNDNPSLKSRVTISVDTSKNQFALKLSSVTAADTAVYYCARERGYTYGNFDHWGQGTLVTVSS

SEQ ID NO: 53 - protein, 246 aa, Artificial Sequence
  Synthesized
DVVMTQTPLSLPVRLGDQASISCRSSQSLVHSNGNTYLHWYLQKPGQSPKLLIYKVSNRFSGVPDRFSGSGSGTNFTLKISRVEAEDLGLYFCSQSTHVPYTFGGGTKLEIKRAGGGGSGGGGSGGGGSQVQLRQSGPELVKPGASVKMSCKASGYTFTDYVISWVKQRTGQGLEWIGDIYPGSGYSFYNENFKGKATLTADKSSTTAYMQLSSLTSEDSAVYFCATYYNYPFAYWGQGTLVTVSA

SEQ ID NO: 54 - protein, 196 aa, Artificial Sequence
  Synthesized
QLVKSELEEKKSELRHKLKYVPHEYIELIEIARNSTQDRILEMKVMEFFMKVYGYRGKHLGGSRKPDGAIYTVGSPIDYGVIVDTKAYSGGYNLPIGQADEMERYVEENQTRNKHLNPNEWWKVYPSSVTEFKFLFVSGHFKGNYKAQLTRLNHITNCNGAVLSVEELLIGGEMIKAGTLTLEEVRRKFNNGEINF

SEQ ID NO: 55 - protein, 242 aa, Artificial Sequence
  Synthesized
DIQMTQSPSSLSASVGDRVTITCRASQDISKYLNWYQQKPGKAPKLLIYHTSRLHSGVPSRFSGSGSGTDFTLTISSLQPEDFATYYCQQGNTLPYTFGQGTKVEIKGGGGSGGGGSGGGGSEVQLVESGGGLVQPGGSLRLSCAASGVSLPDYGVSWVRQAPGKGLEWVSVIWGSETTYYNSALKSRFTISRDNAKNSLYLQMNSLRAEDTAVYYCAKHYYYGGSYAMDYWGQGTLVTVSS

SEQ ID NO: 56 - protein, 199 aa, Artificial Sequence
  Synthesized
LPICPGGAARCQVTLRDLFDRAVVLSHYIHNLSSEMFSEFDKRYTHGRGFITKAINSCHTSSLATPEDKEQAQQMNQKDFLSLIVSILRSWNEPLYHLVTEVRGMQEAPEAILSKAVEIEEQTKRLLEGMELIVSQVHPETKENEIYPVWSGLPSLQMADEESRLSAYYNLLHCLRRDSHKIDNYLKLLKCRIIHNNNC

SEQ ID NO: 57 - protein, 240 aa, Artificial Sequence
  Synthesized
DIVMTQSPDSLAVSLGERATINCKSSQSLLNSRTRKNYLAWYQQKPGQPPKLLIYWASTRESGVPDRFSGSGSGTDFTLTISSLQAEDVAVYYCTQSFILRTFGQGTKVEIKGGGGGSGGGGSGGGGSDIVMTQSPDSLAVSLGERATINCKSSQSLLNSRTRKNYLAWYQQKPGQPPKLLIYWASTRESGVPDRFSGSGSGTDFTLTISSLQAEDVAVYYCTQSFILRTFGQGTKVEIK

SEQ ID NO: 58 - protein, 281 aa, Artificial Sequence
  Synthesized
MNVPTQLLGLLLLWLTGGKCDIQMTQSPASLSASLEEIVTITCKASQAIDAYLSWYQQKPGKSPQLLIYDATSLADGVPSRFSGSRSGTQYSLKISRPQVDDSGIYYCLQSYSTPFTFGSGTKLEIKGGGGGSGGGGSGGGGSMAVLVLLLCLLIFPSCVLSQVQLKESGPGLVQPSQTLSLTCTVSGSSLTSNSVSWIRQPPGKGLEWMGVIWSNGDADYNSAIKSRLSISRDTSKSQVFLKMNSLQTEDTAMYFCASPYYGYYFPFDYWGQGVMVTVSS

SEQ ID NO: 59 - protein, 285 aa, Artificial Sequence
  Synthesized
METDTLLLWVLLLWVPGSTGDIVLTQSPALAVSLGQRATISCRASQSVSISSHDLMQWYQQKPGQQPKLLIYDAFNLASGIPVRFSGSGSGTDFTLTIDPVQADDIATYYCQQSKDDPYTFGAGTKLELKGGGGGSGGGGSGGGGSMDIRLSLAFLVLFIKGVQCEVQLVESGGGLVQPGRSMKLSCAASGFTFSNYGMAWVRQAPTKGLEWVATISYDGSITYYRDSVKGRFTISRDHAKSTLYLQMNSLRSEDTATYYCTREEQYSSWYFDFWGPGIMVTVSS

SEQ ID NO: 60 - protein, 100 aa, Homo sapiens
DGNEEMGGITQTPYKVSISGTTVILTCPQYPGSEILWQHNDKNIGGDEDDKNIGSDEDHLSLKEFSELEQSGYYVCYPRGSKPEDANFYLYLRARVCENC

SEQ ID NO: 61 - protein, 371 aa, Homo sapiens
KKVVLGKKGDTVELTCTASQKKSIQFHWKNSNQIKILGNQGSFLTKGPSKLNDRADSRRSLWDQGNFPLIIKNLKIEDSDTYICEVEDQKEEVQLLVFGLTANSDTHLLQGQSLTLTLESPPGSSPSVQCRSPRGKNIQGGKTLSVSQLELQDSGTWTCTVLQNQKKVEFKIDIVVLAFQKASSIVYKKEGEQVEFSFPLAFTVEKLTGSGELWWQAERASSSKSWITFDLKNKEVSVKRVTQDPKLQMGKKLPLHLTLPQALPQYAGSGNLTLALEAKTGKLHQEVNLVVMRATQLQKNLTCEVWGPTSPKLMLSLKLENKEAKVSKREKAVWVLNPEAGMWQCLLSDSGQVLLESNIKVLPTWSTPVQP

SEQ ID NO: 62 - protein, 348 aa, Homo sapiens
RLSWYDPDFQARLTRSNSKCQGQLEVYLKDGWHMVCSQSWGRSSKQWEDPSQASKVCQRLNCGVPLSLGPFLVTYTPQSSIICYGQLGSFSNCSHSRNDMCHSLGLTCLEPQKTTPPTTRPPPTTTPEPTAPPRLQLVAQSGGQHCAGVVEFYSGSLGGTISYEAQDKTQDLENFLCNNLQCGSFLKHLPETEAGRAQDPGEPREHQPLPIQWKIQNSSCTSLEHCFRKIKPQKSGRVLALLCSGFQPKVQSRLVGGSSICEGTVEVRQGAQWAALCDSSSARSSLRWEEVCREQQCGSVNSYRVLDAGDPTSRGLFCPHQKLSQCHELWERNSYCKKVFVTCQDPNP

SEQ ID NO: 63 - DNA, 7902 bp, Artificial Sequence; identical to SEQ ID NO: 8
  Synthesized

SEQ ID NO: 64 - protein, 66 aa, Artificial Sequence
  Synthesized
TTTPAPRPPTPAPTIASQPLSLRPEACRPAAGGAVHTRGLDFACDIYIWAPLAGTCGVLLLSLVIT

SEQ ID NO: 65 - protein, 69 aa, Artificial Sequence; identical to SEQ ID NO: 35
  Synthesized

SEQ ID NO: 66 - protein, 72 aa, Artificial Sequence
  Synthesized
AKPTTTPAPRPPTPAPTIASQPLSLRPEACRPAAGGAVHTRGLDFACDIYIWAPLAGTCGVLLLSLVITLYC

SEQ ID NO: 67 - protein, 69 aa, Artificial Sequence
  Synthesized
AKPTTTPAPRPPTPAPTIASQPLSLRPEACRPAAGGAVHTRGLDFACDIYIWAPLAGTCGVLLLSLVIT

SEQ ID NO: 68 - protein, 50 aa, Artificial Sequence
  Synthesized
AKPTTTPAPRPPTPAPTIASQPLSLRPEACRPAAGGAVHTRGLDFACDIY

SEQ ID NO: 69 - protein, 50 aa, Artificial Sequence; identical to SEQ ID NO: 68
  Synthesized

SEQ ID NO: 70 - protein, 47 aa, Artificial Sequence; identical to SEQ ID NO: 36
  Synthesized

SEQ ID NO: 71 - protein, 47 aa, Artificial Sequence; identical to SEQ ID NO: 36
  Synthesized

SEQ ID NO: 72 - protein, 22 aa, Artificial Sequence
  Synthesized
IWAPLAGTCGVLLLSLVITLYC

SEQ ID NO: 73 - protein, 19 aa, Artificial Sequence
  Synthesized
IWAPLAGTCGVLLLSLVIT

SEQ ID NO: 74 - protein, 19 aa, Artificial Sequence
  Synthesized
IWAPLAGTCGVLLLSLVIT

SEQ ID NO: 75 - protein, 22 aa, Artificial Sequence
  Synthesized
IWAPLAGTCGVLLLSLVITLYC

SEQ ID NO: 76 - protein, 15 aa, Artificial Sequence
  Synthesized
GGGGSGGGGSGGGGS

SEQ ID NO: 77 - protein, 7 aa, Artificial Sequence
  Synthesized
QWGTRYR

SEQ ID NO: 78 - protein, 7 aa, Artificial Sequence
  Synthesized
QSGDLTR

SEQ ID NO: 79 - protein, 7 aa, Artificial Sequence
  Synthesized
RSDNLRE

SEQ ID NO: 80 - protein, 7 aa, Artificial Sequence
  Synthesized
ERGTLAR

SEQ ID NO: 81 - DNA, 19 bp, Homo sapiens
gttgctccaggccacagca

SEQ ID NO: 82 - protein, 7 aa, Artificial Sequence
  Synthesized
WRSSLAS

SEQ ID NO: 83 - protein, 7 aa, Artificial Sequence
  Synthesized
QSGSLTR

SEQ ID NO: 84 - protein, 7 aa, Artificial Sequence
  Synthesized
DRSNLTR

SEQ ID NO: 85 - DNA, 12 bp, Homo sapiens
gactttgcatgt

SEQ ID NO: 86 - protein, 7 aa, Artificial Sequence
  Synthesized
HKWVLRQ

SEQ ID NO: 87 - protein, 7 aa, Artificial Sequence
  Synthesized
TSGALTR

SEQ ID NO: 88 - protein, 112 aa, Artificial Sequence
  Synthesized
DIVMTQSPDSLAVSLGERATINCKSSQSLLNSRTRKNYLAWYQQKPGQPPKLLIYWASTRESGVPDRFSGSGSGTDFTLTISSLQAEDVAVYYCTQSFILRTFGQGTKVEIK

SEQ ID NO: 89 - protein, 119 aa, Artificial Sequence
  Synthesized
EVQLVQSGAEVKKPGASVKVSCKASGYTFTNYYIHWVRQAPGQGLEWIGWIYPGDGNTKYNEKFKGRATLTADTSTSTAYLELSSLRSEDTAVYYCARDSYSNYYFDYWGQGTLVTVSS

SEQ ID NO: 90 - protein, 127 aa, Artificial Sequence
  Synthesized
MNVPTQLLGLLLLWLTGGKCDIQMTQSPASLSASLEEIVTITCKASQAIDAYLSWYQQKPGKSPQLLIYDATSLADGVPSRFSGSRSGTQYSLKISRPQVDDSGIYYCLQSYSTPFTFGSGTKLEIK

SEQ ID NO: 91 - protein, 138 aa, Artificial Sequence
  Synthesized
MAVLVLLLCLLIFPSCVLSQVQLKESGPGLVQPSQTLSLTCTVSGSSLTSNSVSWIRQPPGKGLEWMGVIWSNGDADYNSAIKSRLSISRDTSKSQVFLKMNSLQTEDTAMYFCASPYYGYYFPFDYWGQGVMVTVSS

SEQ ID NO: 92 - protein, 130 aa, Artificial Sequence
  Synthesized
METDTLLLWVLLLWVPGSTGDIVLTQSPALAVSLGQRATISCRASQSVSISSHDLMQWYQQKPGQQPKLLIYDAFNLASGIPVRFSGSGSGTDFTLTIDPVQADDIATYYCQQSKDDPYTFGAGTKLELK

SEQ ID NO: 93 - protein, 139 aa, Artificial Sequence
  Synthesized
MDIRLSLAFLVLFIKGVQCEVQLVESGGGLVQPGRSMKLSCAASGFTFSNYGMAWVRQAPTKGLEWVATISYDGSITYYRDSVKGRFTISRDHAKSTLYLQMNSLRSEDTATYYCTREEQYSSWYFDFWGPGIMVTVSS

SEQ ID NO: 94 - protein, 242 aa, Artificial Sequence
  Synthesized
NIVMTQSPSSLSASVGDRVTITCQASQDVGTAVAWYQQKPDQSPKLLIYWTSTRHTGVPDRFTGSGSGTDFTLTISSLQPEDIATYFCHQYNSYNTFGSGTKLEIKGGGGGSGGGGSGGGGSQVTLKESGPVLVKPTETLTLTCTFSGFSLSTSGMGVGWIRQAPGKGLEWVAHIWWDDDVYYNPSLKSRLTITKDASKDQVSLKLSSVTAADTAVYYCVRRRATGTGFDYWGQGTLVTVSS

SEQ ID NO: 95 - protein, 106 aa, Artificial Sequence
  Synthesized
NIVMTQSPSSLSASVGDRVTITCQASQDVGTAVAWYQQKPDQSPKLLIYWTSTRHTGVPDRFTGSGSGTDFTLTISSLQPEDIATYFCHQYNSYNTFGSGTKLEIK

SEQ ID NO: 96 - protein, 120 aa, Artificial Sequence
  Synthesized
QVTLKESGPVLVKPTETLTLTCTFSGFSLSTSGMGVGWIRQAPGKGLEWVAHIWWDDDVYYNPSLKSRLTITKDASKDQVSLKLSSVTAADTAVYYCVRRRATGTGFDYWGQGTLVTVSS